European Patent Application EP 4 112 731 A1, published January 4, 2023. Title: System for high-level rAAV production. Applicant: Charité-Universitätsmedizin Berlin, DE. The sequence listing filed with the application follows.

SEQUENCE LISTING (14 sequences)

SEQ ID NO: 1 - DNA, 4679 bp, Adeno-associated virus - 2
  AAV-2 genome
  misc_feature 1..145: /note="left inverted terminal repeat "
  promoter 191..320: /note="p5 promoter region "
  promoter 287: /note="p5 transcription start site"
  gene 321..1906: /gene="rep68 gene"
  gene 321..2183: /gene="rep78 gene"
  promoter 873: /note="p19 transcription start site"
  gene 993..1906: /gene="rep40 gene"
  gene 993..2183: /gene="rep52 gene"
  promoter 1701..1853: /note="p40 promoter"
  misc_feature 1701..2186: /note="RIS-Ad"
  misc_feature 1906: /note="splice donor site "
  misc_feature 2201: /note="minor splice acceptor site "
  gene 2203..4407: /gene="VP open reading frame"
  gene 2203..4407: /gene="VP1 gene"
  misc_feature 2228: /note="major splice acceptor site"
  misc_feature 2228..2249: /note="Rep68/Rep40-s"
  gene 2614..4407: /gene="VP2 gene"
  gene 2809..4407: /gene="VP3 gene"
  misc_feature 4535..4679: /note="right inverted terminal repeat "
ttggccactccctctctgcgcgctcgctcgctcactgaggccgggcgaccaaaggtcgcccgacgcccgggctttgcccgggcggcctcagtgagcgagcgagcgcgcagagagggagtggccaactccatcactaggggttcctggaggggtggagtcgtgacgtgaattacgtcatagggttagggaggtcctgtattagaggtcacgtgagtgttttgcgacattttgcgacaccatgtggtcacgctgggtatttaagcccgagtgagcacgcagggtctccattttgaagcgggaggtttgaacgcgcagccgccatgccggggttttacgagattgtgattaaggtccccagcgaccttgacgggcatctgcccggcatttctgacagctttgtgaactgggtggccgagaaggaatgggagttgccgccagattctgacatggatctgaatctgattgagcaggcacccctgaccgtggccgagaagctgcagcgcgactttctgacggaatggcgccgtgtgagtaaggccccggaggcccttttctttgtgcaatttgagaagggagagagctacttccacatgcacgtgctcgtggaaaccaccggggtgaaatccatggttttgggacgtttcctgagtcagattcgcgaaaaactgattcagagaatttaccgcgggatcgagccgactttgccaaactggttcgcggtcacaaagaccagaaatggcgccggaggcgggaacaaggtggtggatgagtgctacatccccaattacttgctccccaaaacccagcctgagctccagtgggcgtggactaatatggaacagtatttaagcgcctgtttgaatctcacggagcgtaaacggttggtggcgcagcatctgacgcacgtgtcgcagacgcaggagcagaacaaagagaatcagaatcccaattctgatgcgccggtgatcagatcaaaaacttcagccaggtacatggagctggtcgggtggctcgtggacaaggggattacctcggagaagcagtggatccaggaggaccaggcctcatacatctccttcaatgcggcctccaactcgcggtcccaaatcaaggctgccttggacaatgcgggaaagattatgagcctgactaaaaccgcccccgactacctggtgggccagcagcccgtggaggacatttccagcaatcggatttataaaattttggaactaaacgggtacgatccccaatatgcggcttccgtctttctgggatgggccacgaaaaagttcggcaagaggaacaccatctggctgtttgggcctgcaactaccgggaagaccaacatcgcggaggccatagcccacactgtgcccttctacgggtgcgtaaactggaccaatgagaactttcccttcaacgactgtgtcgacaagatggtgatctggtgggaggaggggaagatgaccgccaaggtcgtggagtcggccaaagccattctcggaggaagcaaggtgcgcgtggaccagaaatgcaagtcctcggcccagatagacccgactcccgtgatcgtcacctccaacaccaacatgtgcgccgtgattgacgggaactcaacgaccttcgaacaccagcagccgttgcaagaccggatgttcaaatttgaactcacccgccgtctggatcatgactttgggaaggtcaccaagcaggaagtcaaagactttttccggtgggcaaaggatcacgtggttgaggtggagcatgaattctacgtcaaaaagggtggagccaagaaaagacccgcccccagtgacgcagatataagtgagcccaaacgggtgcgcgagtcagttgcgcagccatcgacgtcagacgcggaagcttcgatcaactacgcagacaggtaccaaaacaaatgttctcgtcacgtgggcatgaatctgatgctgtttccctgcagacaatgcgagagaatgaatcagaattcaaatatctgcttcactcacggacagaaagactgtttagagtgctttcccgtgtcagaatctcaacccgtttctgtcgtcaaaaaggcgtatcagaaactgtgctacattcatcatatcatgggaaaggtgccagacgcttgcactgcctgcgatctggtcaatgtggatttggatgactgcatctttgaacaataaatgatttaaatcaggtatggctgccgatggttatcttccagattggctcgaggacactctctctgaaggaataagacagtggtggaagctcaaacctggcccaccaccaccaaagcccgcagagcggcataaggacgacagcaggggtcttgtgcttcctgggtacaagtacctcggacccttcaacggactcgacaagggagagccggtcaacgaggcagacgccgcggccctcgagcacgacaaagcctacgaccggcagctcgacagcggagacaacccgtacctcaagtacaaccacgccgacgcggagtttcaggagcgccttaaagaagatacgtcttttgggggcaacctcggacgagcagtcttccaggcgaaaaagagggttcttgaacctctgggcctggttgaggaacctgttaagacggctccgggaaaaaagaggccggtagagcactctcctgtggagccagactcctcctcgggaaccggaaaggcgggccagcagcctgcaagaaaaagattgaattttggtcagactggagacgcagactcagtacctgacccccagcctctcggacagccaccagcagccccctctggtctgggaactaatacgatggctacaggcagtggcgcaccaatggcagacaataacgagggcgccgacggagtgggtaattcctcgggaaattggcattgcgattccacatggatgggcgacagagtcatcaccaccagcacccgaacctgggccctgcccacctacaacaaccacctctacaaacaaatttccagccaatcaggagcctcgaacgacaatcactactttggctacagcaccccttgggggtattttgacttcaacagattccactgccacttttcaccacgtgactggcaaagactcatcaacaacaactggggattccgacccaagagactcaacttcaagctctttaacattcaagtcaaagaggtcacgcagaatgacggtacgacgacgattgccaataaccttaccagcacggttcaggtgtttactgactcggagtaccagctcccgtacgtcctcggctcggcgcatcaaggatgcctcccgccgttcccagcagacgtcttcatggtgccacagtatggatacctcaccctgaacaacgggagtcaggcagtaggacgctcttcattttactgcctggagtactttccttctcagatgctgcgtaccggaaacaactttaccttcagctacacttttgaggacgttcctttccacagcagctacgctcacagccagagtctggaccgtctcatgaatcctctcatcgaccagtacctgtattacttgagcagaacaaacactccaagtggaaccaccacgcagtcaaggcttcagttttctcaggccggagcgagtgacattcgggaccagtctaggaactggcttcctggaccctgttaccgccagcagcgagtatcaaagacatctgcggataacaacaacagtgaatactcgtggactggagctaccaagtaccacctcaatggcagagactctctggtgaatccgggcccggccatggcaagccacaaggacgatgaagaaaagttttttcctcagagcggggttctcatctttgggaagcaaggctcagagaaaacaaatgtggacattgaaaaggtcatgattacagacgaagaggaaatcaggacaaccaatcccgtggctacggagcagtatggttctgtatctaccaacctccagagaggcaacagacaagcagctaccgcagatgtcaacacacaaggcgttcttccaggcatggtctggcaggacagagatgtgtaccttcaggggcccatctgggcaaagattccacacacggacggacattttcacccctctcccctcatgggtggattcggacttaaacaccctcctccacagattctcatcaagaacaccccggtacctgcgaatccttcgaccaccttcagtgcggcaaagtttgcttccttcatcacacagtactccacgggacaggtcagcgtggagatcgagtgggagctgcagaaggaaaacagcaaacgctggaatcccgaaattcagtacacttccaactacaacaagtctgttaatgtggactttactgtggacactaatggcgtgtattcagagcctcgccccattggcaccagatacctgactcgtaatctgtaattgcttgttaatcaataaaccgtttaattcgtttcagttgaactttggtctctgcgtatttctttcttatctagtttccatggctacgtagataagtagcatggcgggttaatcattaactacaaggaacccctagtgatggagttggccactccctctctgcgcgctcgctcgctcactgaggccgggcgaccaaaggtcgcccgacgcccgggctttgcccgggcggcctcagtgagcgagcgagcgcgcagagagggagtggccaa

SEQ ID NO: 2 - DNA, 486 bp, Adeno-associated virus - 2
  RIS-Ad
gtcaccaagcaggaagtcaaagactttttccggtgggcaaaggatcacgtggttgaggtggagcatgaattctacgtcaaaaagggtggagccaagaaaagacccgcccccagtgacgcagatataagtgagcccaaacgggtgcgcgagtcagttgcgcagccatcgacgtcagacgcggaagcttcgatcaactacgcagacaggtaccaaaacaaatgttctcgtcacgtgggcatgaatctgatgctgtttccctgcagacaatgcgagagaatgaatcagaattcaaatatctgcttcactcacggacagaaagactgtttagagtgctttcccgtgtcagaatctcaacccgtttctgtcgtcaaaaaggcgtatcagaaactgtgctacattcatcatatcatgggaaaggtgccagacgcttgcactgcctgcgatctggtcaatgtggatttggatgactgcatctttgaacaataa

SEQ ID NO: 3 - DNA, 486 bp, Artificial Sequence
  Recoded RIS-Ad
gtgacgaaacaggaggtgaaggacttctttagatgggccaaggaccacgtggtggaggtcgagcacgagttttatgtgaagaaggggggggccaaaaagcgccctgcaccttccgacgccgacatttccgagccaaagagagtgcgtgagagtgtggcccaaccctccaccagtgatgccgaggcctccattaattatgccgaccgctatcagaataagtgctcaaggcatgtcgggatgaacctgatgctgttcccatgccgccagtgcgagcgcatgaaccagaacagcaacatttgttttacccacgggcagaaggattgcctggaatgcttcccggtcagcgagtcacagccggtgtccgtggtgaagaaagcctaccaaaagctgtgttacatccaccacattatggggaaagtccccgatgcctgtaccgcatgcgacctggtgaacgttgacctcgacgactgcattttcgagcagtaa

SEQ ID NO: 4 - DNA, 135 bp, Artificial Sequence
  sRep (recoded AAV-2 nucleotides 1782 to 1916)
aaggggggggccaaaaagcgccctgcaccttccgacgccgacatttccgagccaaagagagtgcgtgagagtgtggcccaaccctccaccagtgatgccgaggcctccattaattatgccgaccgctatcagaat

SEQ ID NO: 5 - protein, 621 aa, Adeno-associated virus - 2
  Rep78 aa sequence
MPGFYEIVIKVPSDLDGHLPGISDSFVNWVAEKEWELPPDSDMDLNLIEQAPLTVAEKLQRDFLTEWRRVSKAPEALFFVQFEKGESYFHMHVLVETTGVKSMVLGRFLSQIREKLIQRIYRGIEPTLPNWFAVTKTRNGAGGGNKVVDECYIPNYLLPKTQPELQWAWTNMEQYLSACLNLTERKRLVAQHLTHVSQTQEQNKENQNPNSDAPVIRSKTSARYMELVGWLVDKGITSEKQWIQEDQASYISFNAASNSRSQIKAALDNAGKIMSLTKTAPDYLVGQQPVEDISSNRIYKILELNGYDPQYAASVFLGWATKKFGKRNTIWLFGPATTGKTNIAEAIAHTVPFYGCVNWTNENFPFNDCVDKMVIWWEEGKMTAKVVESAKAILGGSKVRVDQKCKSSAQIDPTPVIVTSNTNMCAVIDGNSTTFEHQQPLQDRMFKFELTRRLDHDFGKVTKQEVKDFFRWAKDHVVEVEHEFYVKKGGAKKRPAPSDADISEPKRVRESVAQPSTSDAEASINYADRYQNKCSRHVGMNLMLFPCRQCERMNQNSNICFTHGQKDCLECFPVSESQPVSVVKKAYQKLCYIHHIMGKVPDACTACDLVNVDLDDCIFEQ

SEQ ID NO: 6 - DNA, 245 bp, Herpes simplex virus unknown type
  HSV-TK promoter
ctgcttcatccccgtggcccgttgctcgcgtttgctggcggtgtccccggaagaaatatatttgcatgtctttagttctatgatgacacaaaccccgcccagcgtcttgtcattggcgaattcgaacacgcagatgcagtcggggcggcgcggtcccaggtccacttcgcatattaaggtgacgcgtgtggcctcgaacaccgagcgaccctgcagcgacccgcttaacagcgtcaacagcgtgc

SEQ ID NO: 7 - DNA, 34946 bp, Artificial Sequence
  rep-rAdV nucleic acid sequence
  misc_feature 355..27115: /note="Adenovirus type 5 genome, E1 and E3 deleted"
  variation 25831: /note="not clearly determined"
  misc_feature 27997..28099: /note="right inverted terminal repeats"
  rep_origin 28303..28970: /note="pBR322 origin"
  gene 29779..30570: /gene="kanamycin resistance gene"
  misc_feature 31038..31140: /note="left inverted terminal repeat"
  misc_feature 31220..31368: /note="encapsidation signal"
  misc_feature 31408..31539: /note="sRep recoded sequence in C-terminus of sRep-Stop531"
  gene 31411..33000: /gene="sRep1/531"
  TATA_signal 32472..32478: /note="TATA Box p19 Promoter"
  promoter 33010..33254: /note="HSV-TK promoter"
gtcacctgctctacggcatctcgatccagcatatctcctcgtttcgcgggttggggcggctttcgctgtacggcagtagtcggtgctcgtccagacgggccagggtcatgtctttccacgggcgcagggtcctcgtcagcgtagtctgggtcacggtgaaggggtgcgctccgggctgcgcgctggccagggtgcgcttgaggctggtcctgctggtgctgaagcgctgccggtcttcgccctgcgcgtcggccaggtagcatttgaccatggtgtcatagtccagcccctccgcggcgtggcccttggcgcgcagcttgcccttggaggaggcgccgcacgaggggcagtgcagacttttgagggcgtagagcttgggcgcgagaaataccgattccggggagtaggcatccgcgccgcaggccccgcagacggtctcgcattccacgagccaggtgagctctggccgttcggggtcaaaaaccaggtttcccccatgctttttgatgcgtttcttacctctggtttccatgagccggtgtccacgctcggtgacgaaaaggctgtccgtgtccccgtatacagacttgagaggcctgtcctcgagcggtgttccgcggtcctcctcgtatagaaactcggaccactctgagacaaaggctcgcgtccaggccagcacgaaggaggctaagtgggaggggtagcggtcgttgtccactagggggtccactcgctccagggtgtgaagacacatgtcgccctcttcggcatcaaggaaggtgattggtttgtaggtgtaggccacgtgaccgggtgttcctgaaggggggctataaaagggggtgggggcgcgttcgtcctcactctcttccgcatcgctgtctgcgagggccagctgttggggtgagtactccctctgaaaagcgggcatgacttctgcgctaagattgtcagtttccaaaaacgaggaggatttgatattcacctggcccgcggtgatgcctttgagggtggccgcatccatctggtcagaaaagacaatctttttgttgtcaagcttggtggcaaacgacccgtagagggcgttggacagcaacttggcgatggagcgcagggtttggtttttgtcgcgatcggcgcgctccttggccgcgatgtttagctgcacgtattcgcgcgcaacgcaccgccattcgggaaagacggtggtgcgctcgtcgggcaccaggtgcacgcgccaaccgcggttgtgcagggtgacaaggtcaacgctggtggctacctctccgcgtaggcgctcgttggtccagcagaggcggccgcccttgcgcgagcagaatggcggtagggggtctagctgcgtctcgtccggggggtctgcgtccacggtaaagaccccgggcagcaggcgcgcgtcgaagtagtctatcttgcatccttgcaagtctagcgcctgctgccatgcgcgggcggcaagcgcgcgctcgtatgggttgagtgggggaccccatggcatggggtgggtgagcgcggaggcgtacatgccgcaaatgtcgtaaacgtagaggggctctctgagtattccaagatatgtagggtagcatcttccaccgcggatgctggcgcgcacgtaatcgtatagttcgtgcgagggagcgaggaggtcgggaccgaggttgctacgggcgggctgctctgctcggaagactatctgcctgaagatggcatgtgagttggatgatatggttggacgctggaagacgttgaagctggcgtctgtgagacctaccgcgtcacgcacgaaggaggcgtaggagtcgcgcagcttgttgaccagctcggcggtgacctgcacgtctagggcgcagtagtccagggtttccttgatgatgtcatacttatcctgtcccttttttttccacagctcgcggttgaggacaaactcttcgcggtctttccagtactcttggatcggaaacccgtcggcctccgaacggtaagagcctagcatgtagaactggttgacggcctggtaggcgcagcatcccttttctacgggtagcgcgtatgcctgcgcggccttccggagcgaggtgtgggtgagcgcaaaggtgtccctgaccatgactttgaggtactggtatttgaagtcagtgtcgtcgcatccgccctgctcccagagcaaaaagtccgtgcgctttttggaacgcggatttggcagggcgaaggtgacatcgttgaagagtatctttcccgcgcgaggcataaagttgcgtgtgatgcggaagggtcccggcacctcggaacggttgttaattacctgggcggcgagcacgatctcgtcaaagccgttgatgttgtggcccacaatgtaaagttccaagaagcgcgggatgcccttgatggaaggcaattttttaagttcctcgtaggtgagctcttcaggggagctgagcccgtgctctgaaagggcccagtctgcaagatgagggttggaagcgacgaatgagctccacaggtcacgggccattagcatttgcaggtggtcgcgaaaggtcctaaactggcgacctatggccattttttctggggtgatgcagtagaaggtaagcgggtcttgttcccagcggtcccatccaaggttcgcggctaggtctcgcgcggcagtcactagaggctcatctccgccgaacttcatgaccagcatgaagggcacgagctgcttcccaaaggcccccatccaagtataggtctctacatcgtaggtgacaaagagacgctcggtgcgaggatgcgagccgatcgggaagaactggatctcccgccaccaattggaggagtggctattgatgtggtgaaagtagaagtccctgcgacgggccgaacactcgtgctggcttttgtaaaaacgtgcgcagtactggcagcggtgcacgggctgtacatcctgcacgaggttgacctgacgaccgcgcacaaggaagcagagtgggaatttgagcccctcgcctggcgggtttggctggtggtcttctacttcggctgcttgtccttgaccgtctggctgctcgaggggagttacggtggatcggaccaccacgccgcgcgagcccaaagtccagatgtccgcgcgcggcggtcggagcttgatgacaacatcgcgcagatgggagctgtccatggtctggagctcccgcggcgtcaggtcaggcgggagctcctgcaggtttacctcgcatagacgggtcagggcgcgggctagatccaggtgatacctaatttccaggggctggttggtggcggcgtcgatggcttgcaagaggccgcatccccgcggcgcgactacggtaccgcgcggcgggcggtgggccgcgggggtgtccttggatgatgcatctaaaagcggtgacgcgggcgagcccccggaggtagggggggctccggacccgccgggagagggggcaggggcacgtcggcgccgcgcgcgggcaggagctggtgctgcgcgcgtaggttgctggcgaacgcgacgacgcggcggttgatctcctgaatctggcgcctctgcgtgaagacgacgggcccggtgagcttgagcctgaaagagagttcgacagaatcaatttcggtgtcgttgacggcggcctggcgcaaaatctcctgcacgtctcctgagttgtcttgataggcgatctcggccatgaactgctcgatctcttcctcctggagatctccgcgtccggctcgctccacggtggcggcgaggtcgttggaaatgcgggccatgagctgcgagaaggcgttgaggcctccctcgttccagacgcggctgtagaccacgcccccttcggcatcgcgggcgcgcatgaccacctgcgcgagattgagctccacgtgccgggcgaagacggcgtagtttcgcaggcgctgaaagaggtagttgagggtggtggcggtgtgttctgccacgaagaagtacataacccagcgtcgcaacgtggattcgttgatatcccccaaggcctcaaggcgctccatggcctcgtagaagtccacggcgaagttgaaaaactgggagttgcgcgccgacacggttaactcctcctccagaagacggatgagctcggcgacagtgtcgcgcacctcgcgctcaaaggctacaggggcctcttcttcttcttcaatctcctcttccataagggcctccccttcttcttcttctggcggcggtgggggaggggggacacggcggcgacgacggcgcaccgggaggcggtcgacaaagcgctcgatcatctccccgcggcgacggcgcatggtctcggtgacggcgcggccgttctcgcgggggcgcagttggaagacgccgcccgtcatgtcccggttatgggttggcggggggctgccatgcggcagggatacggcgctaacgatgcatctcaacaattgttgtgtaggtactccgccgccgagggacctgagcgagtccgcatcgaccggatcggaaaacctctcgagaaaggcgtctaaccagtcacagtcgcaaggtaggctgagcaccgtggcgggcggcagcgggcggcggtcggggttgtttctggcggaggtgctgctgatgatgtaattaaagtaggcggtcttgagacggcggatggtcgacagaagcaccatgtccttgggtccggcctgctgaatgcgcaggcggtcggccatgccccaggcttcgttttgacatcggcgcaggtctttgtagtagtcttgcatgagcctttctaccggcacttcttcttctccttcctcttgtcctgcatctcttgcatctatcgctgcggcggcggcggagtttggccgtaggtggcgccctcttcctcccatgcgtgtgaccccgaagcccctcatcggctgaagcagggctaggtcggcgacaacgcgctcggctaatatggcctgctgcacctgcgtgagggtagactggaagtcatccatgtccacaaagcggtggtatgcgcccgtgttgatggtgtaagtgcagttggccataacggaccagttaacggtctggtgacccggctgcgagagctcggtgtacctgagacgcgagtaagccctcgagtcaaatacgtagtcgttgcaagtccgcaccaggtactggtatcccaccaaaaagtgcggcggcggctggcggtagaggggccagcgtagggtggccggggctccgggggcgagatcttccaacataaggcgatgatatccgtagatgtacctggacatccaggtgatgccggcggcggtggtggaggcgcgcggaaagtcgcggacgcggttccagatgttgcgcagcggcaaaaagtgctccatggtcgggacgctctggccggtcaggcgcgcgcaatcgttgacgctctaccgtgcaaaaggagagcctgtaagcgggcactcttccgtggtctggtggataaattcgcaagggtatcatggcggacgaccggggttcgagccccgtatccggccgtccgccgtgatccatgcggttaccgcccgcgtgtcgaacccaggtgtgcgacgtcagacaacgggggagtgctccttttggcttccttccaggcgcggcggctgctgcgctagcttttttggccactggccgcgcgcagcgtaagcggttaggctggaaagcgaaagcattaagtggctcgctccctgtagccggagggttattttccaagggttgagtcgcgggacccccggttcgagtctcggaccggccggactgcggcgaacgggggtttgcctccccgtcatgcaagaccccgcttgcaaattcctccggaaacagggacgagccccttttttgcttttcccagatgcatccggtgctgcggcagatgcgcccccctcctcagcagcggcaagagcaagagcagcggcagacatgcagggcaccctcccctcctcctaccgcgtcaggaggggcgacatccgcggttgacgcggcagcagatggtgattacgaacccccgcggcgccgggcccggcactacctggacttggaggagggcgagggcctggcgcggctaggagcgccctctcctgagcggtacccaagggtgcagctgaagcgtgatacgcgtgaggcgtacgtgccgcggcagaacctgtttcgcgaccgcgagggagaggagcccgaggagatgcgggatcgaaagttccacgcagggcgcgagctgcggcatggcctgaatcgcgagcggttgctgcgcgaggaggactttgagcccgacgcgcgaaccgggattagtcccgcgcgcgcacacgtggcggccgccgacctggtaaccgcatacgagcagacggtgaaccaggagattaactttcaaaaaagctttaacaaccacgtgcgtacgcttgtggcgcgcgaggaggtggctataggactgatgcatctgtgggactttgtaagcgcgctggagcaaaacccaaatagcaagccgctcatggcgcagctgttccttatagtgcagcacagcagggacaacgaggcattcagggatgcgctgctaaacatagtagagcccgagggccgctggctgctcgatttgataaacatcctgcagagcatagtggtgcaggagcgcagcttgagcctggctgacaaggtggccgccatcaactattccatgcttagcctgggcaagttttacgcccgcaagatataccataccccttacgttcccatagacaaggaggtaaagatcgaggggttctacatgcgcatggcgctgaaggtgcttaccttgagcgacgacctgggcgtttatcgcaacgagcgcatccacaaggccgtgagcgtgagccggcggcgcgagctcagcgaccgcgagctgatgcacagcctgcaaagggccctggctggcacgggcagcggcgatagagaggccgagtcctactttgacgcgggcgctgacctgcgctgggccccaagccgacgcgccctggaggcagctggggccggacctgggctggcggtggcacccgcgcgcgctggcaacgtcggcggcgtggaggaatatgacgaggacgatgagtacgagccagaggacggcgagtactaagcggtgatgtttctgatcagatgatgcaagacgcaacggacccggcggtgcgggcggcgctgcagagccagccgtccggccttaactccacggacgactggcgccaggtcatggaccgcatcatgtcgctgactgcgcgcaatcctgacgcgttccggcagcagccgcaggccaaccggctctccgcaattctggaagcggtggtcccggcgcgcgcaaaccccacgcacgagaaggtgctggcgatcgtaaacgcgctggccgaaaacagggccatccggcccgacgaggccggcctggtctacgacgcgctgcttcagcgcgtggctcgttacaacagcggcaacgtgcagaccaacctggaccggctggtgggggatgtgcgcgaggccgtggcgcagcgtgagcgcgcgcagcagcagggcaacctgggctccatggttgcactaaacgccttcctgagtacacagcccgccaacgtgccgcggggacaggaggactacaccaactttgtgagcgcactgcggctaatggtgactgagacaccgcaaagtgaggtgtaccagtctgggccagactattttttccagaccagtagacaaggcctgcagaccgtaaacctgagccaggctttcaaaaacttgcaggggctgtggggggtgcgggctcccacaggcgaccgcgcgaccgtgtctagcttgctgacgcccaactcgcgcctgttgctgctgctaatagcgcccttcacggacagtggcagcgtgtcccgggacacatacctaggtcacttgctgacactgtaccgcgaggccataggtcaggcgcatgtggacgagcatactttccaggagattacaagtgtcagccgcgcgctggggcaggaggacacgggcagcctggaggcaaccctaaactacctgctgaccaaccggcggcagaagatcccctcgttgcacagtttaaacagcgaggaggagcgcattttgcgctacgtgcagcagagcgtgagccttaacctgatgcgcgacggggtaacgcccagcgtggcgctggacatgaccgcgcgcaacatggaaccgggcatgtatgcctcaaaccggccgtttatcaaccgcctaatggactacttgcatcgcgcggccgccgtgaaccccgagtatttcaccaatgccatcttgaacccgcactggctaccgccccctggtttctacaccgggggattcgaggtgcccgagggtaacgatggattcctctgggacgacatagacgacagcgtgttttccccgcaaccgcagaccctgctagagttgcaacagcgcgagcaggcagaggcggcgctgcgaaaggaaagcttccgcaggccaagcagcttgtccgatctaggcgctgcggccccgcggtcagatgctagtagcccatttccaagcttgatagggtctcttaccagcactcgcaccacccgcccgcgcctgctgggcgaggaggagtacctaaacaactcgctgctgcagccgcagcgcgaaaaaaacctgcctccggcatttcccaacaacgggatagagagcctagtggacaagatgagtagatggaagacgtacgcgcaggagcacagggacgtgccaggcccgcgcccgcccacccgtcgtcaaaggcacgaccgtcagcggggtctggtgtgggaggacgatgactcggcagacgacagcagcgtcctggatttgggagggagtggcaacccgtttgcgcaccttcgccccaggctggggagaatgttttaaaaaaaaaaaagcatgatgcaaaataaaaaactcaccaaggccatggcaccgagcgttggttttcttgtattccccttagtatgcggcgcgcggcgatgtatgaggaaggtcctcctccctcctacgagagtgtggtgagcgcggcgccagtggcggcggcgctgggttctcccttcgatgctcccctggacccgccgtttgtgcctccgcggtacctgcggcctaccggggggagaaacagcatccgttactctgagttggcacccctattcgacaccacccgtgtgtacctggtggacaacaagtcaacggatgtggcatccctgaactaccagaacgaccacagcaactttctgaccacggtcattcaaaacaatgactacagcccgggggaggcaagcacacagaccatcaatcttgacgaccggtcgcactggggcggcgacctgaaaaccatcctgcataccaacatgccaaatgtgaacgagttcatgtttaccaataagtttaaggcgcgggtgatggtgtcgcgcttgcctactaaggacaatcaggtggagctgaaatacgagtgggtggagttcacgctgcccgagggcaactactccgagaccatgaccatagaccttatgaacaacgcgatcgtggagcactacttgaaagtgggcagacagaacggggttctggaaagcgacatcggggtaaagtttgacacccgcaacttcagactggggtttgaccccgtcactggtcttgtcatgcctggggtatatacaaacgaagccttccatccagacatcattttgctgccaggatgcggggtggacttcacccacagccgcctgagcaacttgttgggcatccgcaagcggcaacccttccaggagggctttaggatcacctacgatgatctggagggtggtaacattcccgcactgttggatgtggacgcctaccaggcgagcttgaaagatgacaccgaacagggcgggggtggcgcaggcggcagcaacagcagtggcagcggcgcggaagagaactccaacgcggcagccgcggcaatgcagccggtggaggacatgaacgatcatgccattcgcggcgacacctttgccacacgggctgaggagaagcgcgctgaggccgaagcagcggccgaagctgccgcccccgctgcgcaacccgaggtcgagaagcctcagaagaaaccggtgatcaaacccctgacagaggacagcaagaaacgcagttacaacctaataagcaatgacagcaccttcacccagtaccgcagctggtaccttgcatacaactacggcgaccctcagaccggaatccgctcatggaccctgctttgcactcctgacgtaacctgcggctcggagcaggtctactggtcgttgccagacatgatgcaagaccccgtgaccttccgctccacgcgccagatcagcaactttccggtggtgggcgccgagctgttgcccgtgcactccaagagcttctacaacgaccaggccgtctactcccaactcatccgccagtttacctctctgacccacgtgttcaatcgctttcccgagaaccagattttggcgcgcccgccagcccccaccatcaccaccgtcagtgaaaacgttcctgctctcacagatcacgggacgctaccgctgcgcaacagcatcggaggagtccagcgagtgaccattactgacgccagacgccgcacctgcccctacgtttacaaggccctgggcatagtctcgccgcgcgtcctatcgagccgcactttttgagcaagcatgtccatccttatatcgcccagcaataacacaggctggggcctgcgcttcccaagcaagatgtttggcggggccaagaagcgctccgaccaacacccagtgcgcgtgcgcgggcactaccgcgcgccctggggcgcgcacaaacgcggccgcactgggcgcaccaccgtcgatgacgccatcgacgcggtggtggaggaggcgcgcaactacacgcccacgccgccaccagtgtccacagtggacgcggccattcagaccgtggtgcgcggagcccggcgctatgctaaaatgaagagacggcggaggcgcgtagcacgtcgccaccgccgccgacccggcactgccgcccaacgcgcggcggcggccctgcttaaccgcgcacgtcgcaccggccgacgggcggccatgcgggccgctcgaaggctggccgcgggtattgtcactgtgccccccaggtccaggcgacgagcggccgccgcagcagccgcggccattagtgctatgactcagggtcgcaggggcaacgtgtattgggtgcgcgactcggttagcggcctgcgcgtgcccgtgcgcacccgccccccgcgcaactagattgcaagaaaaaactacttagactcgtactgttgtatgtatccagcggcggcggcgcgcaacgaagctatgtccaagcgcaaaatcaaagaagagatgctccaggtcatcgcgccggagatctatggccccccgaagaaggaagagcaggattacaagccccgaaagctaaagcgggtcaaaaagaaaaagaaagatgatgatgatgaacttgacgacgaggtggaactgctgcacgctaccgcgcccaggcgacgggtacagtggaaaggtcgacgcgtaaaacgtgttttgcgacccggcaccaccgtagtctttacgcccggtgagcgctccacccgcacctacaagcgcgtgtatgatgaggtgtacggcgacgaggacctgcttgagcaggccaacgagcgcctcggggagtttgcctacggaaagcggcataaggacatgctggcgttgccgctggacgagggcaacccaacacctagcctaaagcccgtaacactgcagcaggtgctgcccgcgcttgcaccgtccgaagaaaagcgcggcctaaagcgcgagtctggtgacttggcacccaccgtgcagctgatggtacccaagcgccagcgactggaagatgtcttggaaaaaatgaccgtggaacctgggctggagcccgaggtccgcgtgcggccaatcaagcaggtggcgccgggactgggcgtgcagaccgtggacgttcagatacccactaccagtagcaccagtattgccaccgccacagagggcatggagacacaaacgtccccggttgcctcagcggtggcggatgccgcggtgcaggcggtcgctgcggccgcgtccaagacctctacggaggtgcaaacggacccgtggatgtttcgcgtttcagccccccggcgcccgcgcggttcgaggaagtacggcgccgccagcgcgctactgcccgaatatgccctacatccttccattgcgcctacccccggctatcgtggctacacctaccgccccagaagacgagcaactacccgacgccgaaccaccactggaacccgccgccgccgtcgccgtcgccagcccgtgctggccccgatttccgtgcgcagggtggctcgcgaaggaggcaggaccctggtgctgccaacagcgcgctaccaccccagcatcgtttaaaagccggtctttgtggttcttgcagatatggccctcacctgccgcctccgtttcccggtgccgggattccgaggaagaatgcaccgtaggaggggcatggccggccacggcctgacgggcggcatgcgtcgtgcgcaccaccggcggcggcgcgcgtcgcaccgtcgcatgcgcggcggtatcctgcccctccttattccactgatcgccgcggcgattggcgccgtgcccggaattgcatccgtggccttgcaggcgcagagacactgattaaaaacaagttgcatgtggaaaaatcaaaataaaaagtctggactctcacgctcgcttggtcctgtaactattttgtagaatggaagacatcaactttgcgtctctggccccgcgacacggctcgcgcccgttcatgggaaactggcaagatatcggcaccagcaatatgagcggtggcgccttcagctggggctcgctgtggagcggcattaaaaatttcggttccaccgttaagaactatggcagcaaggcctggaacagcagcacaggccagatgctgagggataagttgaaagagcaaaatttccaacaaaaggtggtagatggcctggcctctggcattagcggggtggtggacctggccaaccaggcagtgcaaaataagattaacagtaagcttgatccccgccctcccgtagaggagcctccaccggccgtggagacagtgtctccagaggggcgtggcgaaaagcgtccgcgccccgacagggaagaaactctggtgacgcaaatagacgagcctccctcgtacgaggaggcactaaagcaaggcctgcccaccacccgtcccatcgcgcccatggctaccggagtgctgggccagcacacacccgtaacgctggacctgcctccccccgccgacacccagcagaaacctgtgctgccaggcccgaccgccgttgttgtaacccgtcctagccgcgcgtccctgcgccgcgccgccagcggtccgcgatcgttgcggcccgtagccagtggcaactggcaaagcacactgaacagcatcgtgggtctgggggtgcaatccctgaagcgccgacgatgcttctgaatagctaacgtgtcgtatgtgtgtcatgtatgcgtccatgtcgccgccagaggagctgctgagccgccgcgcgcccgctttccaagatggctaccccttcgatgatgccgcagtggtcttacatgcacatctcgggccaggacgcctcggagtacctgagccccgggctggtgcagtttgcccgcgccaccgagacgtacttcagcctgaataacaagtttagaaaccccacggtggcgcctacgcacgacgtgaccacagaccggtcccagcgtttgacgctgcggttcatccctgtggaccgtgaggatactgcgtactcgtacaaggcgcggttcaccctagctgtgggtgataaccgtgtgctggacatggcttccacgtactttgacatccgcggcgtgctggacaggggccctacttttaagccctactctggcactgcctacaacgccctggctcccaagggtgccccaaatccttgcgaatgggatgaagctgctactgctcttgaaataaacctagaagaagaggacgatgacaacgaagacgaagtagacgagcaagctgagcagcaaaaaactcacgtatttgggcaggcgccttattctggtataaatattacaaaggagggtattcaaataggtgtcgaaggtcaaacacctaaatatgccgataaaacatttcaacctgaacctcaaataggagaatctcagtggtacgaaactgaaattaatcatgcagctgggagagtccttaaaaagactaccccaatgaaaccatgttacggttcatatgcaaaacccacaaatgaaaatggagggcaaggcattcttgtaaagcaacaaaatggaaagctagaaagtcaagtggaaatgcaatttttctcaactactgaggcgaccgcaggcaatggtgataacttgactcctaaagtggtattgtacagtgaagatgtagatatagaaaccccagacactcatatttcttacatgcccactattaaggaaggtaactcacgagaactaatgggccaacaatctatgcccaacaggcctaattacattgcttttagggacaattttattggtctaatgtattacaacagcacgggtaatatgggtgttctggcgggccaagcatcgcagttgaatgctgttgtagatttgcaagacagaaacacagagctttcataccagcttttgcttgattccattggtgatagaaccaggtacttttctatgtggaatcaggctgttgacagctatgatccagatgttagaattattgaaaatcatggaactgaagatgaacttccaaattactgctttccactgggaggtgtgattaatacagagactcttaccaaggtaaaacctaaaacaggtcaggaaaatggatgggaaaaagatgctacagaattttcagataaaaatgaaataagagttggaaataattttgccatggaaatcaatctaaatgccaacctgtggagaaatttcctgtactccaacatagcgctgtatttgcccgacaagctaaagtacagtccttccaacgtaaaaatttctgataacccaaacacctacgactacatgaacaagcgagtggtggctcccgggttagtggactgctacattaaccttggagcacgctggtcccttgactatatggacaacgtcaacccatttaaccaccaccgcaatgctggcctgcgctaccgctcaatgttgctgggcaatggtcgctatgtgcccttccacatccaggtgcctcagaagttctttgccattaaaaacctccttctcctgccgggctcatacacctacgagtggaacttcaggaaggatgttaacatggttctgcagagctccctaggaaatgacctaagggttgacggagccagcattaagtttgatagcatttgcctttacgccaccttcttccccatggcccacaacaccgcctccacgcttgaggccatgcttagaaacgacaccaacgaccagtcctttaacgactatctctccgccgccaacatgctctaccctatacccgccaacgctaccaacgtgcccatatccatcccctcccgcaactgggcggctttccgcggctgggccttcacgcgccttaagactaaggaaaccccatcactgggctcgggctacgacccttattacacctactctggctctataccctacctagatggaaccttttacctcaaccacacctttaagaaggtggccattacctttgactcttctgtcagctggcctggcaatgaccgcctgcttacccccaacgagtttgaaattaagcgctcagttgacggggagggttacaacgttgcccagtgtaacatgaccaaagactggttcctggtacaaatgctagctaactacaacattggctaccagggcttctatatcccagagagctacaaggaccgcatgtactccttctttagaaacttccagcccatgagccgtcaggtggtggatgatactaaatacaaggactaccaacaggtgggcatcctacaccaacacaacaactctggatttgttggctaccttgcccccaccatgcgcgaaggacaggcctaccctgctaacttcccctatccgcttataggcaagaccgcagttgacagcattacccagaaaaagtttctttgcgatcgcaccctttggcgcatcccattctccagtaactttatgtccatgggcgcactcacagacctgggccaaaaccttctctacgccaactccgcccacgcgctagacatgacttttgaggtggatcccatggacgagcccacccttctttatgttttgtttgaagtctttgacgtggtccgtgtgcaccggccgcaccgcggcgtcatcgaaaccgtgtacctgcgcacgcccttctcggccggcaacgccacaacataaagaagcaagcaacatcaacaacagctgccgccatgggctccagtgagcaggaactgaaagccattgtcaaagatcttggttgtgggccatattttttgggcacctatgacaagcgctttccaggctttgtttctccacacaagctcgcctgcgccatagtcaatacggccggtcgcgagactgggggcgtacactggatggcctttgcctggaacccgcactcaaaaacatgctacctctttgagccctttggcttttctgaccagcgactcaagcaggtttaccagtttgagtacgagtcactcctgcgccgtagcgccattgcttcttcccccgaccgctgtataacgctggaaaagtccacccaaagcgtacaggggcccaactcggccgcctgtggactattctgctgcatgtttctccacgcctttgccaactggccccaaactcccatggatcacaaccccaccatgaaccttattaccggggtacccaactccatgctcaacagtccccaggtacagcccaccctgcgtcgcaaccaggaacagctctacagcttcctggagcgccactcgccctacttccgcagccacagtgcgcagattaggagcgccacttctttttgtcacttgaaaaacatgtaaaaataatgtactagagacactttcaataaaggcaaatgcttttatttgtacactctcgggtgattatttacccccacccttgccgtctgcgccgtttaaaaatcaaaggggttctgccgcgcatcgctatgcgccactggcagggacacgttgcgatactggtgtttagtgctccacttaaactcaggcacaaccatccgcggcagctcggtgaagttttcactccacaggctgcgcaccatcaccaacgcgtttagcaggtcgggcgccgatatcttgaagtcgcagttggggcctccgccctgcgcgcgcgagttgcgatacacagggttgcagcactggaacactatcagcgccgggtggtgcacgctggccagcacgctcttgtcggagatcagatccgcgtccaggtcctccgcgttgctcagggcgaacggagtcaactttggtagctgccttcccaaaaagggcgcgtgcccaggctttgagttgcactcgcaccgtagtggcatcaaaaggtgaccgtgcccggtctgggcgttaggatacagcgcctgcataaaagccttgatctgcttaaaagccacctgagcctttgcgccttcagagaagaacatgccgcaagacttgccggaaaactgattggccggacaggccgcgtcgtgcacgcagcaccttgcgtcggtgttggagatctgcaccacatttcggccccaccggttcttcacgatcttggccttgctagactgctccttcagcgcgcgctgcccgttttcgctcgtcacatccatttcaatcacgtgctccttatttatcataatgcttccgtgtagacacttaagctcgccttcgatctcagcgcagcggtgcagccacaacgcgcagcccgtgggctcgtgatgcttgtaggtcacctctgcaaacgactgcaggtacgcctgcaggaatcgccccatcatcgtcacaaaggtcttgttgctggtgaaggtcagctgcaacccgcggtgctcctcgttcagccaggtcttgcatacggccgccagagcttccacttggtcaggcagtagtttgaagttcgcctttagatcgttatccacgtggtacttgtccatcagcgcgcgcgcagcctccatgcccttctcccacgcagacacgatcggcacactcagcgggttcatcaccgtaatttcactttccgcttcgctgggctcttcctcttcctcttgcgtccgcataccacgcgccactgggtcgtcttcattcagccgccgcactgtgcgcttacctcctttgccatgcttgattagcaccggtgggttgctgaaacccaccatttgtagcgccacatcttctctttcttcctcgctgtccacgattacctctggtgatggcgggcgctcgggcttgggagaagggcgcttctttttcttcttgggcgcaatggccaaatccgccgccgaggtcgatggccgcgggctgggtgtgcgcggcaccagcgcgtcttgtgatgagtcttcctcgtcctcggactcgatacgccgcctcatccgcttttttgggggcgcccggggaggcggcggcgacggggacggggacgacacgtcctccatggttgggggacgtcgcgccgcaccgcgtccgcgctcgggggtggtttcgcgctgctcctcttcccgactggccatttccttctcctataggcagaaaaagatcatggagtcagtcgagaagaaggacagcctaaccgccccctctgagttcgccaccaccgcctccaccgatgccgccaacgcgcctaccaccttccccgtcgaggcacccccgcttgaggaggaggaagtgattatcgagcaggacccaggttttgtaagcgaagacgacgaggaccgctcagtaccaacagaggataaaaagcaagaccaggacaacgcagaggcaaacgaggaacaagtcgggcggggggacgaaaggcatggcgactacctagatgtgggagacgacgtgctgttgaagcatctgcagcgccagtgcgccattatctgcgacgcgttgcaagagcgcagcgatgtgcccctcgccatagcggatgtcagccttgcctacgaacgccacctattctcaccgcgcgtaccccccaaacgccaagaaaacggcacatgcgagcccaacccgcgcctcaacttctaccccgtatttgccgtgccagaggtgcttgccacctatcacatctttttccaaaactgcaagatacccctatcctgccgtgccaaccgcagccgagcggacaagcagctggccttgcggcagggcgctgtcatacctgatatcgcctcgctcaacgaagtgccaaaaatctttgagggtcttggacgcgacgagaagcgcgcggcaaacgctctgcaacaggaaaacagcgaaaatgaaagtcactctggagtgttggtggaactcgagggtgacaacgcgcgcctagccgtactaaaacgcagcatcgaggtcacccactttgcctacccggcacttaacctaccccccaaggtcatgagcacagtcatgagtgagctgatcgtgcgccgtgcgcagcccctggagagggatgcaaatttgcaagaacaaacagaggagggcctacccgcagttggcgacgagcagctagcgcgctggcttcaaacgcgcgagcctgccgacttggaggagcgacgcaaactaatgatggccgcagtgctcgttaccgtggagcttgagtgcatgcagcggttctttgctgacccggagatgcagcgcaagctagaggaaacattgcactacacctttcgacagggctacgtacgccaggcctgcaagatctccaacgtggagctctgcaacctggtctcctaccttggaattttgcacgaaaaccgccttgggcaaaacgtgcttcattccacgctcaagggcgaggcgcgccgcgactacgtccgcgactgcgtttacttatttctatgctacacctggcagacggccatgggcgtttggcagcagtgcttggaggagtgcaacctcaaggagctgcagaaactgctaaagcaaaacttgaaggacctatggacggccttcaacgagcgctccgtggccgcgcacctggcggacatcattttccccgaacgcctgcttaaaaccctgcaacagggtctgccagacttcaccagtcaaagcatgttgcagaactttaggaactttatcctagagcgctcaggaatcttgcccgccacctgctgtgcacttcctagcgactttgtgcccattaagtaccgcgaatgccctccgccgctttggggccactgctaccttctgcagctagccaactaccttgcctaccactctgacataatggaagacgtgagcggtgacggtctactggagtgtcactgtcgctgcaacctatgcaccccgcaccgctccctggtttgcaattcgcagctgcttaacgaaagtcaaattatcggtacctttgagctgcagggtccctcgcctgacgaaaagtccgcggctccggggttgaaactcactccggggctgtggacgtcggcttaccttcgcaaatttgtacctgaggactaccacgcccacgagattaggttctacgaagaccaatcccgcccgccaaatgcggagcttaccgcctgcgtcattacccagggccacattcttggccaattgcaagccatcaacaaagcccgccaagagtttctgctacgaaagggacggggggtttacttggacccccagtccggcgaggagctcaacccaatccccccgccgccgcagccctatcagcagcagccgcgggcccttgcttcccaggatggcacccaaaaagaagctgcagctgccgccgccacccacggacgaggaggaatactgggacagtcaggcagaggaggttttggacgaggaggaggaggacatgatggaagactgggagagcctagacgaggaagcttccgaggtcgaagaggtgtcagacgaaacaccgtcaccctcggtcgcattcccctcgccggcgccccagaaatcggcaaccggttccagcatggctacaacctccgctcctcaggcgccgccggcactgcccgttcgccgacccaaccgtagatgggacaccactggaaccagggccggtaagtccaagcagccgccgccgttagcccaagagcaacaacagcgccaaggctaccgctcatggcgcgggcacaagaacgccatagttgcttgcttgcaagactgtgggggcaacatctccttcgcccgccgctttcttctctaccatcacggcgtggccttcccccgtaacatcctgcattactaccgtcatctctacagcccatactgcaccggcggcagcggcagcggcagcaacagcagcggccacacagaagcaaaggcgaccggatagcaagactctgacaaagcccaagaaatccacagcggcggcagcagcaggaggaggagcgctgcgtctggcgcccaacgaacccgtatcgacccgcgagcttagaaacaggatttttcccactctgtatgctatatttcaacagagcaggggccaagaacaagagctgaaaataaaaaacaggtctctgcgatccctcacccgcagctgcctgtatcacaaaagcgaagatcagcttcggcgcacgctggaagacgcggaggctctcttcagtaaatactgcgcgctgactcttaaggactagtttcgcgccctttctcaaatttaagcgcgaaaactacgtcatctccagcggccacacccggcgccagcacctgtcgtcagcgccattatgagcaaggaaattcccacgccctacatgtggagttaccagccacaaatgggacttgcggctggagctgcccaagactactcaacccgaataaactacatgagcgcgggaccccacatgatatcccgggtcaacggaatccgcgcccaccgaaaccgaattctcttggaacaggcggctattaccaccacacctcgtaataaccttaatccccgtagttggcccgctgccctggtgtaccaggaaagtcccgctcccaccactgtggtacttcccagagacgcccaggccgaagttcagatgactaactcaggggcgcagcttgcgggcggctttcgtcacagggtgcggtcgcccgggcagggtataactcacctgacaatcagagggcgaggtattcagctcaacgacgagtcggtgagctcctcgcttggtctccgtccggacgggacatttcagatcggcggcgccggccgtccttcattcacgcctcgtcaggcaatcctaactctgcagacctcgtcctctgagccgcgctctggaggcattggaactctgcaatttattgaggagtttgtgccatcggtctactttaaccccttctcgggacctcccggccactatccggatcaatttattcctaactttgacgcggtaaaggactcggcggacggctacgactgaatgttaagtggagaggcagagcaactgcgcctgaaacacctggtccactgtcgccgccacaagtgctttgcccgcgactccggtgagttttgctactttgaattgcccgaggatcatatcgagggcccggcgcacggcgtccggcttaccgcccagggagagcttgcccgtagcctgattcgggagtttacccagcgccccctgctagttgagcgggacaggggaccctgtgttctcactgtgatttgcaactgtcctaaccttggattacatcaagatcctctagttataactagagtacccggggatcttattccctttaactaataaaaaaaaataataaagcatcacttacttaaaatcagttagcaaatttctgtccagtttattcagcagcacctccttgccctcctcccagctctggtattgcagcttcctcctggctgcaaactttctccacaatctaaatggaatgtcagtttcctcctgttcctgtccatccgcacccactatcttcatgttgttgcagatgaagcgcgcaagaccgtctgaagataccttcaaccccgtgtatccatatgacacggaaaccggtcctccaactgtgccttttcttactcctccctttgtatcccccaatgggtttcaagagagtccccctggggtactctctttgcgcctatccgaacctctagttacctccaatggcatgcttgcgctcaaaatgggcaacggcctctctctggacgaggccggcaaccttacctcccaaaatgtaaccactgtgagcccacctctcaaaaaaaccaagtcaaacataaacctggaaatatctgcacccctcacagttacctcagaagccctaactgtggctgccgccgcacctctaatggtcgcgggcaacacactcaccatgcaatcacaggccccgctaaccgtgcacgactccaaacttagcattgccacccaaggacccctcacagtgtcagaaggaaagctagccctgcaaacatcaggccccctcaccaccaccgatagcagtacccttactatcactgcctcaccccctctaactactgccactggtagcttgggcattgacttgaaagagcccatttatacacaaaatggaaaactaggactaaagtacggggctcctttgcatgtaacagacgacctaaacactttgaccgtagcaactggtccaggtgtgactattaataatacttccttgcaaactaaagttactggagccttgggttttgattcacaaggcaatatgcaacttaatgtagcaggaggactaaggattgattctcaaaacagacgccttatacttgatgttagttatccgtttgatgctcaaaaccaactaaatctaagactaggacagggccctctttttataaactcagcccacaacttggatattaactacaacaaaggcctttacttgtttacagcttcaaacaattccaaaaagcttgaggttaacctaagcactgccaaggggttgatgtttgacgctacagccatagccattaatgcaggagatgggcttgaatttggttcacctaatgcaccaaacacaaatcccctcaaaacaaaaattggccatggcctagaatttgattcaaacaaggctatggttcctaaactaggaactggccttagttttgacagcacaggtgccattacagtaggaaacaaaaataatgataagctaactttgtggaccacaccagctccatctcctaactgtagactaaatgcagagaaagatgctaaactcactttggtcttaacaaaatgtggcagtcaaatacttgctacagtttcagttttggctgttaaaggcagtttggctccaatatctggaacagttcaaagtgctcatcttattataagatttgacgaaaatggagtgctactaaacaattccttcctggacccagaatattggaactttagaaatggagatcttactgaaggcacagcctatacaaacgctgttggatttatgcctaacctatcagcttatccaaaatctcacggtaaaactgccaaaagtaacattgtcagtcaagtttacttaaacggagacaaaactaaacctgtaacactaaccattacactaaacggtacacaggaaacaggagacacaactccaagtgcatactctatgtcattttcatgggactggtctggccacaactacattaatgaaatatttgccacatcctcttacactttttcatacattgcccaagaataaagaatcgtttgtgttatgtttcaacgtgtttatttttcaattgcagaaaatttcaagtcatttttcattcagtagtatagccccaccaccacatagcttatacagatcaccgtaccttaatcaaactcacagaaccctagtattcaacctgccacctccctcccaacacacagagtacacagtcctttctccccggctggccttaaaaagcatcatatcatgggtaacagacatattcttaggtgttatattccacacggtttcctgtcgagccaaacgctcatcaagtgatattaataaactccccgggcagctcacttaagttcatgtcgctgtccagctgctgagccacaggctgctgtccaacttgcggttgcttaacgggcggcgaaggagaagtccacgcctacatggggggagagtcataatcgtgcatcaggatagggcggtggtgctgcagcagcgcgcgaataaactgctgccgccgccgctccgtcctgcaggaatacaacatggcagtggtctcctcagcgatgattcgcaccgcccgcagcataaggcgcttgtcctccgggcacagcagcgcaccctgatctcacttaaatcagcacagtaactgcagcacagcaccacaatattgttcaaaatcccacagtgcaaggcgctgtatccaaagctcatggcggggaccacagaacccacgtggccatcataccacaagcgcaggtagattaagtggcgacccctcataaacacgctggacataaacattacctcttttggcatgttgtaattcaccacctcccggtaccatataaacctctgattaaacatggcgccatccaccaccatcctaaaccagctggccaaaacctgccccgccgggntatacactgcagggaaccgggacttggacaatgacaagtgggagagcccaggactcgtaaccatggatcatcatgctcgtcatgatatcaatgttggcacaacacaggcacacgtgcatacacttcctcaggattacaagctcctcccgcgttagaaccatatcccagggaacaacccattcctgaatcagcgtaaatcccacactgcagggaagacctcgcacgtaactcacgttgtgcattgtcaaagtgttacattcgggcagcagcggatgatcctccagtatggtagcgcgggtttctgtctcaaaaggaggtagacgatccctactgtacggagtgcgccgagacaaccgagatcgtgttggtcgtagtgtcatgccaaatggaacgccggacgtagtcatatttcctgaagcaaaaccaggtgcgggcgtgacaaacagatctgcgtctccggtctcgccgcttagatcgctctgtgtagtagttgtagtatatccactctctcaaagcatccaggcgccccctggcttcgggttctatgtaaactccttcatgcgccgctgccctgataacatccaccaccgcagaataagccacacccagccaacctacacattcgttctgcgagtcacacacgggaggagcgggaagagctggaagaaccatgtttttttttttattccaaaagattatccaaaacctcaaaatgaagatctattaagtgaacgcgctcccctccggtggcgtggtcaaactctacagccaaagaacagataatggcatttgtaagatgttgcacaatggcttccaaaaggcaaacggccctcacgtccaagtggacgtaaaggctaaacccttcagggtgaatctcctctataaacattccagcaccttcaaccatgcccaaataattctcatctcgccaccttctcaatatatctctaagcaaatcccgaatatttaagtccgggccattgtaaaaaatttggctccagagcgccctccaccttcagcctcaagcagcgaatcatgattgcaaaaattcaggttcctcacagacctgtataagattcaaaagcggaacattaacaaaaataccgcgatcccgtaggtcccttcgcagggccagctgaacataatcgtgcaggtctgcacggaccagcgcggccacttccccgccaggaaccatgacaaaagaacccacactgattatgacacgcatactcggagctatgctaaccagcgtagccccgatgtaagcttgttgcatgggcggcgatataaaatgcaaggtgctgctcaaaaaatcaggcaaagcctcgcgcaaaaaagaaagcacatcgtagtcatgctcatgcagataaaggcaggtaagctccggaaccaccacagaaaaagacaccatttttctctcaaacatgtctgcgggtttctgcataaacacaaaataaaataacaaaaaaacatttaaacattagaagcctgtcttacaacaggaaaaacaacccttataagcataagacggactacggccatgccggcgtgaccgtaaaaaaactggtcaccgtgattaaaaagcaccaccgacagctcctcggtcatgtccggagtcataatgtaagactcggtaaacacatcaggttgattcatcggtcagtgctaaaaagcgaccgaaatagcccgggggaatacatacccgcaggcgtagagacaacattacagcccccataggaggtataacaaaattaataggagagaaaaacacataaacacctgaaaaaccctcctgcctaggcaaaatagcaccctcccgctccagaacaacatacagcgcttcacagcggcagcctaacagtcagccttaccagtaaaaaagaaaacctattaaaaaaacaccactcgacacggcaccagctcaatcagtcacagtgtaaaaaagggccaagtgcagagcgagtatatataggactaaaaaatgacgtaacggttaaagtccacaaaaaacacccagaaaaccgcacgcgaacctacgcccagaaacgaaagccaaaaaacccacaacttcctcaaatcgtcacttccgttttcccacgttacgtaacttcccattttaagaaaactacaattcccaacacatacaagttactccgccctaaaacctacgtcacccgccccgttcccacgccccgcgccacgtcacaaactccaccccctcattatcatattggcttcaatccaaaataaggtatattattgatgatgttaattaacatgcatggatccatatgcggtgtgaaataccgcacagatgcgtaaggagaaaataccgcatcaggcgctcttccgcttcctcgctcactgactcgctgcgctcggtcgttcggctgcggcgagcggtatcagctcactcaaaggcggtaatacggttatccacagaatcaggggataacgcaggaaagaacatgtgagcaaaaggccagcaaaaggccaggaaccgtaaaaaggccgcgttgctggcgtttttccataggctccgcccccctgacgagcatcacaaaaatcgacgctcaagtcagaggtggcgaaacccgacaggactataaagataccaggcgtttccccctggaagctccctcgtgcgctctcctgttccgaccctgccgcttaccggatacctgtccgcctttctcccttcgggaagcgtggcgctttctcatagctcacgctgtaggtatctcagttcggtgtaggtcgttcgctccaagctgggctgtgtgcacgaaccccccgttcagcccgaccgctgcgccttatccggtaactatcgtcttgagtccaacccggtaagacacgacttatcgccactggcagcagccactggtaacaggattagcagagcgaggtatgtaggcggtgctacagagttcttgaagtggtggcctaactacggctacactagaaggacagtatttggtatctgcgctctgctgaagccagttaccttcggaaaaagagttggtagctcttgatccggcaaacaaaccaccgctggtagcggtggtttttttgtttgcaagcagcagattacgcgcagaaaaaaaggatctcaagaagatcctttgatcttttctacggggtctgacgctcagtggaacgaaaactcacgttaagggattttggtcatgagattatcaaaaaggatcttcacctagatccttttaaattaaaaatgaagttttaaatcaatctaaagtatatatgagtaaacttggtctgacagttaccaatgcttaatcagtgaggcacctatctcagcgatctgtctatttcgttcatccatagttgcctgactccccgtcgtgtagataactacgatacgggagggcttaccatctggccccagtgctgcaatgataccgcgagacccacgctcaccggctccagatttatcagcaataaaccagccagccggaagggccgagcgcagaagtggtcctgcaactttatccgcctccatccagtctattaattgttgccgggaagctagagtaagtagttcgccagttaatagtttgcgcaacgttgttgccattgctgcagccatgagattatcaaaaaggatcttcacctagatccttttcacgtagaaagccagtccgcagaaacggtgctgaccccggatgaatgtcagctactgggctatctggacaagggaaaacgcaagcgcaaagagaaagcaggtagcttgcagtgggcttacatggcgatagctagactgggcggttttatggacagcaagcgaaccggaattgccagctggggcgccctctggtaaggttgggaagccctgcaaagtaaactggatggctttcttgccgccaaggatctgatggcgcaggggatcaagctctgatcaagagacaggatgaggatcgtttcgcatgattgaacaagatggattgcacgcaggttctccggccgcttgggtggagaggctattcggctatgactgggcacaacagacaatcggctgctctgatgccgccgtgttccggctgtcagcgcaggggcgcccggttctttttgtcaagaccgacctgtccggtgccctgaatgaactgcaagacgaggcagcgcggctatcgtggctggccacgacgggcgttccttgcgcagctgtgctcgacgttgtcactgaagcgggaagggactggctgctattgggcgaagtgccggggcaggatctcctgtcatctcaccttgctcctgccgagaaagtatccatcatggctgatgcaatgcggcggctgcatacgcttgatccggctacctgcccattcgaccaccaagcgaaacatcgcatcgagcgagcacgtactcggatggaagccggtcttgtcgatcaggatgatctggacgaagagcatcaggggctcgcgccagccgaactgttcgccaggctcaaggcgagcatgcccgacggcgaggatctcgtcgtgacccatggcgatgcctgcttgccgaatatcatggtggaaaatggccgcttttctggattcatcgactgtggccggctgggtgtggcggaccgctatcaggacatagcgttggctacccgtgatattgctgaagagcttggcggcgaatgggctgaccgcttcctcgtgctttacggtatcgccgctcccgattcgcagcgcatcgccttctatcgccttcttgacgagttcttctgaattttgttaaaatttttgttaaatcagctcattttttaaccaataggccgaaatcggcaacatcccttataaatcaaaagaatagaccgcgatagggttgagtgttgttccagtttggaacaagagtccactattaaagaacgtggactccaacgtcaaagggcgaaaaaccgtctatcagggcgatggcccactacgtgaaccatcacccaaatcaagttttttgcggtcgaggtgccgtaaagctctaaatcggaaccctaaagggagcccccgatttagagcttgacggggaaagccggcgaacgtggcgagaaaggaagggaagaaagcgaaaggagcgggcgctagggcgctggcaagtgtagcggtcacgctgcgcgtaaccaccacacccgcgcgcttaatgcgccgctacagggcgcgtccattcgccattcaggatcgaattaattcttaattaacatcatcaataatataccttattttggattgaagccaatatgataatgagggggtggagtttgtgacgtggcgcggggcgtgggaacggggcgggtgacgtagtagtgtggcggaagtgtgatgttgcaagtgtggcggaacacatgtaagcgacggatgtggcaaaagtgacgtttttggtgtgcgccggtgtacacaggaagtgacaattttcgcgcggttttaggcggatgttgtagtaaatttgggcgtaaccgagtaagatttggccattttcgcgggaaaactgaataagaggaagtgaaatctgaataattttgtgttactcatagcgcgtaatactggtaccgcggccgcctcgagtctagattaatagcggtcggcataattaatggaggcctcggcatcactggtggagggttgggccacactctcacgcactctctttggctcggaaatgtcggcgtcggaaggtgcagggcgctttttggcccccccctttttgacgtagaattcatgctccacctcaaccacgtgatcctttgcccaccggaaaaagtctttgacttcctgcttggtgaccttcccaaagtcatgatccagacggcgggtgagttcaaatttgaacatccggtcttgcaacggctgctggtgttcgaaggtcgttgagttcccgtcaatcacggcgcacatgttggtgttggaggtgacgatcacgggagtcgggtctatctgggccgaggacttgcatttctggtccacgcgcaccttgcttcctccgagaatggctttggccgactccacgaccttggcggtcatcttcccctcctcccaccagatcaccatcttgtcgacacagtcgttgaagggaaagttctcattggtccagtttacgcacccgtagaagggcacagtgtgggctatggcctccgcgatgttggtcttcccggtagttgcaggcccaaacagccagatggtgttcctcttgccgaactttttcgtggcccatcccagaaagacggaagccgcatattggggatcgtacccgtttagttccaaaattttataaatccgattgctggaaatgtcctccacgggctgctggcccaccaggtagtcgggggcggttttagtcaggctcataatctttcccgcattgtccaaggcagccttgatttgggaccgcgagttggaggccgcattgaaggagatgtatgaggcctggtcctcctggatccactgcttctccgaggtaatccccttgtccacgagccacccgaccagctccatgtacctggctgaagtttttgatctgatcaccggcgcatcagaattgggattctgattctctttgttctgctcctgcgtctgcgacacgtgcgtcagatgctgcgccaccaaccgtttacgctccgtgagattcaaacaggcgcttaaatactgttccatattagtccacgcccactggagctcaggctgggttttggggagcaagtaattggggatgtagcactcatccaccaccttgttcccgcctccggcgccatttctggtctttgtgaccgcgaaccagtttggcaaagtcggctcgatcccgcggtaaattctctgaatcagtttttcgcgaatctgactcaggaaacgtcccaaaaccatggatttcaccccggtggtttccacgagcacgtgcatgtggaagtagctctctcccttctcaaattgcacaaagaaaagggcctccggggccttactcacacggcgccattccgtcagaaagtcgcgctgcagcttctcggccacggtcaggggtgcctgctcaatcagattcagatccatgtcagaatctggcggcaactcccattccttctcggccacccagttcacaaagctgtcagaaatgccgggcagatgcccgtcaaggtcgctggggaccttaatcacaatctcgtaaaaccccggcatggcaccggtgcacgctgttgacgctgttaagcgggtcgctgcagggtcgctcggtgttcgaggccacacgcgtcaccttaatatgcgaagtggacctgggaccgcgccgccccgactgcatctgcgtgttcgaattcgccaatgacaagacgctgggcggggtttgtgtcatcatagaactaaagacatgcaaatatatttcttccggggacaccgccagcaaacgcgagcaacgggccacggggatgaagcagactagtcataagcttgtcgactcgaagatctgggcgtggttaagggtgggaaagaatatataaggtgggggtcttatgtagttttgtatctgttttgcagcagccgccgccgccatgagcaccaactcgtttgatggaagcattgtgagctcatatttgacaacgcgcatgcccccatgggccggggtgcgtcagaatgtgatgggctccagcattgatggtcgccccgtcctgcccgcaaactctactaccttgacctacgagaccgtgtctggaacgccgttggagactgcagcctccgccgccgcttcagccgctgcagccaccgcccgcgggattgtgactgactttgctttcctgagcccgcttgcaagcagtgcagcttcccgttcatccgcccgcgatgacaagttgacggctcttttggcacaattggattctttgacccgggaacttaatgtcgtttctcagcagctgttggatctgcgccagcaggtttctgccctgaaggcttcctcccctcccaatgcggtttaaaacataaataaaaaaccagactctgtttggatttggatcaagcaagtgtcttgctgtctttatttaggggttttgcgcgcgcggtaggcccgggaccagcggtctcggtcgttgagggtcctgtgtattttttccaggacgtggtaaaggtgactctggatgttcagatacatgggcataagcccgtctctggggtggaggtagcaccactgcagagcttcatgctgcggggtggtgttgtagatgatccagtcgtagcaggagcgctgggcgtggtgcctaaaaatgtctttcagtagcaagctgattgccaggggcaggcccttggtgtaagtgtttacaaagcggttaagctgggatgggtgcatacgtggggatatgagatgcatcttggactgtatttttaggttggctatgttcccagccatatccctccggggattcatgttgtgcagaaccaccagcacagtgtatccggtgcacttgggaaatttgtcatgtagcttagaaggaaatgcgtggaagaacttggagacgcccttgtgacctccaagattttccatgcattcgtccataatgatggcaatgggcccacgggcggcggcctgggcgaagatatttctgggatcactaacgtcatagttgtgttccaggatgagatcgtcataggccatttttacaaagcgcgggcggagggtgccagactgcggtataatggttccatccggcccaggggcgtagttaccctcacagatttgcatttcccacgctttgagttcagatggggggatcatgtctacctgcggggcgatgaagaaaacggtttccggggtaggggagatcagctgggaagaaagcaggttcctgagcagctgcgacttaccgcagccggtgggcccgtaaatcacacctattaccgggtgcaactggtagttaagagagctgcagctgccgtcatccctgagcaggggggccacttcgttaagcatgtccctgactcgcatgttttccctgaccaaatccgccagaaggcgctcgccgcccagcgatagcagttcttgcaaggaagcaaagtttttcaacggtttgagaccgtccgccgtaggcatgcttttgagcgtttgaccaagcagttccaggcggtcccacagctcg

SEQ ID NO: 8 - DNA, 156 bp, Artificial Sequence
  Recoded p40 promoter 1
gtcaccaagcaggaagtcaaagactttttccggtgggcaaaggatcacgtggttgaggtggagcatgaattctacgtcaaaaaggggggggccaaaaagcgccctgcaccttccgacgccgacatttccgagccaaagagagtgcgtgagagtgtg

SEQ ID NO: 9 - DNA, 156 bp, Artificial Sequence
  Recoded p40 promoter 2
gtcaccaagcaggaagtcaaagactttttccggtgggcaaaggatcacgtggttgaggtggagcatgaattctacgtcaaaaaggggggggccaagaaaagacccgcccccagtgacgcagatataagtgagcccaaacgggtgcgcgagagtgtg

SEQ ID NO: 10 - DNA, 37669 bp, Artificial Sequence
  cap-rAdV nucleic acid sequence
  gene 3330..4121: /gene="kanamycin resistance gene"
  misc_feature 4589..4691: /note="left inverted terminal repeat"
  misc_feature 4771..4919: /note="encapsidation signal"
  promoter 4967..5211: /note="HSV-TK promoter"
  misc_feature 5236: /note="splice donor site"
  misc_feature 5531: /note="minor splice acceptor site"
  gene 5533..7737: /gene="VP open reading frame"
  gene 5533..7737: /gene="VP1 gene"
  misc_feature 5558: /note="major splice acceptor site"
  gene 5944..7737: /gene="VP2 gene"
  gene 6139..7737: /gene="VP3 gene"
  polyA_site 7754..7758: /note="polyadenylation site"
  misc_feature 9920..36680: /note="Ad5 genome (E1/E3 deleted)"
  variation 35396: /note="not clearly determined"
  misc_feature 36681..37669: /note="Ad5 left arm homology"
  variation 37085: /note="not clearly determined"
ttaattaacatgcatggatcctcgtctcgacgatgcccttgagagccttcaacccagtcagctccttccggtgggcgcggggcatgactatcgtcgccgcacttatgactgtcttctttatcatgcaactcgtaggacaggtgccggcagcgctctgggtcattttcggcgaggaccgctttcgctggagcgcgacgatgatcggcctgtcgcttgcggtattcggaatcttgcacgccctcgctcaagccttcgtcactggtcccgccaccaaacgtttcggcgagaagcaggccattatcgccggcatggcggccgacgcgctgggctacgtcttgctggcgttcgcgacgcgaggctggatggccttccccattatgattcttctcgcttccggcggcatcgggatgcccgcgttgcaggccatgctgtccaggcaggtagatgacgaccatcagggacagcttcaaggatcgctcgcggctcttaccagcctaacttcgatcactggaccgctgatcgtcacggcgatttatgccgcctcggcgagcacatggaacgggttggcatggattgtaggcgccgccctataccttgtctgcctccccgcgttgcgtcgcggtgcatggagccgggccacctcgacctgaatggaagccggcggcacctcgctaacggattcaccactccaagaattggagccaatcaattcttgcggagaactgtgaatgcgcaaaccaacccttggcagaacatatccatcgcgtccgccatctccagcagccgcacgcggcgcatctcgggcagcgttgggtcctggccacgggtgcgcatgatcgtgctcctgtcgttgaggacccggctaggctggcggggttgccttactggttagcagaatgaatcaccgatacgcgagcgaacgtgaagcgactgctgctgcaaaacgtctgcgacctgagcaacaacatgaatggtcttcggtttccgtgtttcgtaaagtctggaaacgcggaagtcagcgccctgcaccattatgttccggatctgcatcgcaggatgctgctggctaccctgtggaacacctacatctgtattaacgaagcgctggcattgaccctgagtgatttttctctggtcccgccgcatccataccgccagttgtttaccctcacaacgttccagtaaccgggcatgttcatcatcagtaacccgtatcgtgagcatcctctctcgtttcatcggtatcattacccccatgaacagaaattcccccttacacggaggcatcaagtgaccaaacaggaaaaaaccgcccttaacatggcccgctttatcagaagccagacattaacgcttctggagaaactcaacgagctggacgcggatgaacaggcagacatctgtgaatcgcttcacgaccacgctgatgagctttaccgcagctgcctcgcgcgtttcggtgatgacggtgaaaacctctgacacatgcagctcccggagacggtcacagcttgtctgtaagcggatgccgggagcagacaagcccgtcagggcgcgtcagcgggtgttggcgggtgtcggggcgcagccatgacccagtcacgtagcgatagcggagtgtatactggcttaactatgcggcatcagagcagattgtactgagagtgcaccatatgcggtgtgaaataccgcacagatgcgtaaggagaaaataccgcatcaggcgctcttccgcttcctcgctcactgactcgctgcgctcggtcgttcggctgcggcgagcggtatcagctcactcaaaggcggtaatacggttatccacagaatcaggggataacgcaggaaagaacatgtgagcaaaaggccagcaaaaggccaggaaccgtaaaaaggccgcgttgctggcgtttttccataggctccgcccccctgacgagcatcacaaaaatcgacgctcaagtcagaggtggcgaaacccgacaggactataaagataccaggcgtttccccctggaagctccctcgtgcgctctcctgttccgaccctgccgcttaccggatacctgtccgcctttctcccttcgggaagcgtggcgctttctcaatgctcacgctgtaggtatctcagttcggtgtaggtcgttcgctccaagctgggctgtgtgcacgaaccccccgttcagcccgaccgctgcgccttatccggtaactatcgtcttgagtccaacccggtaagacacgacttatcgccactggcagcagccactggtaacaggattagcagagcgaggtatgtaggcggtgctacagagttcttgaagtggtggcctaactacggctacactagaaggacagtatttggtatctgcgctctgctgaagccagttaccttcggaaaaagagttggtagctcttgatccggcaaacaaaccaccgctggtagcggtggtttttttgtttgcaagcagcagattacgcgcagaaaaaaaggatctcaagaagatcctttgatcttttctacggggtctgacgctcagtggaacgaaaactcacgttaagggattttggtcatgagattatcaaaaaggatcttcacctagatccttttaaattaaaaatgaagttttaaatcaatctaaagtatatatgagtaaacttggtctgacagttaccaatgcttaatcagtgaggcacctatctcagcgatctgtctatttcgttcatccatagttgcctgactccccgtcgtgtagataactacgatacgggagggcttaccatctggccccagtgctgcaatgataccgcgagacccacgctcaccggctccagatttatcagcaataaaccagccagccggaagggccgagcgcagaagtggtcctgcaactttatccgcctccatccagtctattaattgttgccgggaagctagagtaagtagttcgccagttaatagtttgcgcaacgttgttgccattgctgcagccatgagattatcaaaaaggatcttcacctagatccttttcacgtagaaagccagtccgcagaaacggtgctgaccccggatgaatgtcagctactgggctatctggacaagggaaaacgcaagcgcaaagagaaagcaggtagcttgcagtgggcttacatggcgatagctagactgggcggttttatggacagcaagcgaaccggaattgccagctggggcgccctctggtaaggttgggaagccctgcaaagtaaactggatggctttcttgccgccaaggatctgatggcgcaggggatcaagctctgatcaagagacaggatgaggatcgtttcgcatgattgaacaagatggattgcacgcaggttctccggccgcttgggtggagaggctattcggctatgactgggcacaacagacaatcggctgctctgatgccgccgtgttccggctgtcagcgcaggggcgcccggttctttttgtcaagaccgacctgtccggtgccctgaatgaactgcaagacgaggcagcgcggctatcgtggctggccacgacgggcgttccttgcgcagctgtgctcgacgttgtcactgaagcgggaagggactggctgctattgggcgaagtgccggggcaggatctcctgtcatctcaccttgctcctgccgagaaagtatccatcatggctgatgcaatgcggcggctgcatacgcttgatccggctacctgcccattcgaccaccaagcgaaacatcgcatcgagcgagcacgtactcggatggaagccggtcttgtcgatcaggatgatctggacgaagagcatcaggggctcgcgccagccgaactgttcgccaggctcaaggcgagcatgcccgacggcgaggatctcgtcgtgacccatggcgatgcctgcttgccgaatatcatggtggaaaatggccgcttttctggattcatcgactgtggccggctgggtgtggcggaccgctatcaggacatagcgttggctacccgtgatattgctgaagagcttggcggcgaatgggctgaccgcttcctcgtgctttacggtatcgccgctcccgattcgcagcgcatcgccttctatcgccttcttgacgagttcttctgaattttgttaaaatttttgttaaatcagctcattttttaaccaataggccgaaatcggcaacatcccttataaatcaaaagaatagaccgcgatagggttgagtgttgttccagtttggaacaagagtccactattaaagaacgtggactccaacgtcaaagggcgaaaaaccgtctatcagggcgatggcccactacgtgaaccatcacccaaatcaagttttttgcggtcgaggtgccgtaaagctctaaatcggaaccctaaagggagcccccgatttagagcttgacggggaaagccggcgaacgtggcgagaaaggaagggaagaaagcgaaaggagcgggcgctagggcgctggcaagtgtagcggtcacgctgcgcgtaaccaccacacccgcgcgcttaatgcgccgctacagggcgcgtccattcgccattcaggatcgaattaattcttaattaacatcatcaataatataccttattttggattgaagccaatatgataatgagggggtggagtttgtgacgtggcgcggggcgtgggaacggggcgggtgacgtagtagtgtggcggaagtgtgatgttgcaagtgtggcggaacacatgtaagcgacggatgtggcaaaagtgacgtttttggtgtgcgccggtgtacacaggaagtgacaattttcgcgcggttttaggcggatgttgtagtaaatttgggcgtaaccgagtaagatttggccattttcgcgggaaaactgaataagaggaagtgaaatctgaataattttgtgttactcatagcgcgtaatactggtaccgcggccgcctcgagtctagatgactagtctgcttcatccccgtggcccgttgctcgcgtttgctggcggtgtccccggaagaaatatatttgcatgtctttagttctatgatgacacaaaccccgcccagcgtcttgtcattggcgaattcgaacacgcagatgcagtcggggcggcgcggtcccaggtccacttcgcatattaaggtgacgcgtgtggcctcgaacaccgagcgaccctgcagcgacccgcttaacagcgtcaacagcgtgcaagcttcgatcaactacgcagacaggtaccaaaacaaatgttctcgtcacgtgggcatgaatctgatgctgtttccctgcagacaatgcgagagaatgaatcagaattcaaatatctgcttcactcacggacagaaagactgtttagagtgctttcccgtgtcagaatctcaacccgtttctgtcgtcaaaaaggcgtatcagaaactgtgctacattcatcatatcatgggaaaggtgccagacgcttgcactgcctgcgatctggtcaatgtggatttggatgactgcatctttgaacaataaatgatttaaatcaggtatggctgccgatggttatcttccagattggctcgaggacactctctctgaaggaataagacagtggtggaagctcaaacctggcccaccaccaccaaagcccgcagagcggcataaggacgacagcaggggtcttgtgcttcctgggtacaagtacctcggacccttcaacggactcgacaagggagagccggtcaacgaggcagacgccgcggccctcgagcacgacaaagcctacgaccggcagctcgacagcggagacaacccgtacctcaagtacaaccacgccgacgcggagtttcaggagcgccttaaagaagatacgtcttttgggggcaacctcggacgagcagtcttccaggcgaaaaagagggttcttgaacctctgggcctggttgaggaacctgttaagacggctccgggaaaaaagaggccggtagagcactctcctgtggagccagactcctcctcgggaaccggaaaggcgggccagcagcctgcaagaaaaagattgaattttggtcagactggagacgcagactcagtacctgacccccagcctctcggacagccaccagcagccccctctggtctgggaactaatacgatggctacaggcagtggcgcaccaatggcagacaataacgagggcgccgacggagtgggtaattcctcgggaaattggcattgcgattccacatggatgggcgacagagtcatcaccaccagcacccgaacctgggccctgcccacctacaacaaccacctctacaaacaaatttccagccaatcaggagcctcgaacgacaatcactactttggctacagcaccccttgggggtattttgacttcaacagattccactgccacttttcaccacgtgactggcaaagactcatcaacaacaactggggattccgacccaagagactcaacttcaagctctttaacattcaagtcaaagaggtcacgcagaatgacggtacgacgacgattgccaataaccttaccagcacggttcaggtgtttactgactcggagtaccagctcccgtacgtcctcggctcggcgcatcaaggatgcctcccgccgttcccagcagacgtcttcatggtgccacagtatggatacctcaccctgaacaacgggagtcaggcagtaggacgctcttcattttactgcctggagtactttccttctcagatgctgcgtaccggaaacaactttaccttcagctacacttttgaggacgttcctttccacagcagctacgctcacagccagagtctggaccgtctcatgaatcctctcatcgaccagtacctgtattacttgagcagaacaaacactccaagtggaaccaccacgcagtcaaggcttcagttttctcaggccggagcgagtgacattcgggaccagtctaggaactggcttcctggaccctgttaccgccagcagcgagtatcaaagacatctgcggataacaacaacagtgaatactcgtggactggagctaccaagtaccacctcaatggcagagactctctggtgaatccgggcccggccatggcaagccacaaggacgatgaagaaaagttttttcctcagagcggggttctcatctttgggaagcaaggctcagagaaaacaaatgtggacattgaaaaggtcatgattacagacgaagaggaaatcaggacaaccaatcccgtggctacggagcagtatggttctgtatctaccaacctccagagaggcaacagacaagcagctaccgcagatgtcaacacacaaggcgttcttccaggcatggtctggcaggacagagatgtgtaccttcaggggcccatctgggcaaagattccacacacggacggacattttcacccctctcccctcatgggtggattcggacttaaacaccctcctccacagattctcatcaagaacaccccggtacctgcgaatccttcgaccaccttcagtgcggcaaagtttgcttccttcatcacacagtactccacgggacaggtcagcgtggagatcgagtgggagctgcagaaggaaaacagcaaacgctggaatcccgaaattcagtacacttccaactacaacaagtctgttaatgtggactttactgtggacactaatggcgtgtattcagagcctcgccccattggcaccagatacctgactcgtaatctgtaattgcttgttaatcaataaaccgtttaattcgtttcagttgaactttggtctctgcgtatttctttcttatctagtttccatggctacgtagataagtagcatggcgggttaatcattctagctagagatatcgaattcaagctagcttgtcgactcgaagatctgggcgtggttaagggtgggaaagaatatataaggtgggggtcttatgtagttttgtatctgttttgcagcagccgccgccgccatgagcaccaactcgtttgatggaagcattgtgagctcatatttgacaacgcgcatgcccccatgggccggggtgcgtcagaatgtgatgggctccagcattgatggtcgccccgtcctgcccgcaaactctactaccttgacctacgagaccgtgtctggaacgccgttggagactgcagcctccgccgccgcttcagccgctgcagccaccgcccgcgggattgtgactgactttgctttcctgagcccgcttgcaagcagtgcagcttcccgttcatccgcccgcgatgacaagttgacggctcttttggcacaattggattctttgacccgggaacttaatgtcgtttctcagcagctgttggatctgcgccagcaggtttctgccctgaaggcttcctcccctcccaatgcggtttaaaacataaataaaaaaccagactctgtttggatttggatcaagcaagtgtcttgctgtctttatttaggggttttgcgcgcgcggtaggcccgggaccagcggtctcggtcgttgagggtcctgtgtattttttccaggacgtggtaaaggtgactctggatgttcagatacatgggcataagcccgtctctggggtggaggtagcaccactgcagagcttcatgctgcggggtggtgttgtagatgatccagtcgtagcaggagcgctgggcgtggtgcctaaaaatgtctttcagtagcaagctgattgccaggggcaggcccttggtgtaagtgtttacaaagcggttaagctgggatgggtgcatacgtggggatatgagatgcatcttggactgtatttttaggttggctatgttcccagccatatccctccggggattcatgttgtgcagaaccaccagcacagtgtatccggtgcacttgggaaatttgtcatgtagcttagaaggaaatgcgtggaagaacttggagacgcccttgtgacctccaagattttccatgcattcgtccataatgatggcaatgggcccacgggcggcggcctgggcgaagatatttctgggatcactaacgtcatagttgtgttccaggatgagatcgtcataggccatttttacaaagcgcgggcggagggtgccagactgcggtataatggttccatccggcccaggggcgtagttaccctcacagatttgcatttcccacgctttgagttcagatggggggatcatgtctacctgcggggcgatgaagaaaacggtttccggggtaggggagatcagctgggaagaaagcaggttcctgagcagctgcgacttaccgcagccggtgggcccgtaaatcacacctattaccgggtgcaactggtagttaagagagctgcagctgccgtcatccctgagcaggggggccacttcgttaagcatgtccctgactcgcatgttttccctgaccaaatccgccagaaggcgctcgccgcccagcgatagcagttcttgcaaggaagcaaagtttttcaacggtttgagaccgtccgccgtaggcatgcttttgagcgtttgaccaagcagttccaggcggtcccacagctcggtcacctgctctacggcatctcgatccagcatatctcctcgtttcgcgggttggggcggctttcgctgtacggcagtagtcggtgctcgtccagacgggccagggtcatgtctttccacgggcgcagggtcctcgtcagcgtagtctgggtcacggtgaaggggtgcgctccgggctgcgcgctggccagggtgcgcttgaggctggtcctgctggtgctgaagcgctgccggtcttcgccctgcgcgtcggccaggtagcatttgaccatggtgtcatagtccagcccctccgcggcgtggcccttggcgcgcagcttgcccttggaggaggcgccgcacgaggggcagtgcagacttttgagggcgtagagcttgggcgcgagaaataccgattccggggagtaggcatccgcgccgcaggccccgcagacggtctcgcattccacgagccaggtgagctctggccgttcggggtcaaaaaccaggtttcccccatgctttttgatgcgtttcttacctctggtttccatgagccggtgtccacgctcggtgacgaaaaggctgtccgtgtccccgtatacagacttgagaggcctgtcctcgagcggtgttccgcggtcctcctcgtatagaaactcggaccactctgagacaaaggctcgcgtccaggccagcacgaaggaggctaagtgggaggggtagcggtcgttgtccactagggggtccactcgctccagggtgtgaagacacatgtcgccctcttcggcatcaaggaaggtgattggtttgtaggtgtaggccacgtgaccgggtgttcctgaaggggggctataaaagggggtgggggcgcgttcgtcctcactctcttccgcatcgctgtctgcgagggccagctgttggggtgagtactccctctgaaaagcgggcatgacttctgcgctaagattgtcagtttccaaaaacgaggaggatttgatattcacctggcccgcggtgatgcctttgagggtggccgcatccatctggtcagaaaagacaatctttttgttgtcaagcttggtggcaaacgacccgtagagggcgttggacagcaacttggcgatggagcgcagggtttggtttttgtcgcgatcggcgcgctccttggccgcgatgtttagctgcacgtattcgcgcgcaacgcaccgccattcgggaaagacggtggtgcgctcgtcgggcaccaggtgcacgcgccaaccgcggttgtgcagggtgacaaggtcaacgctggtggctacctctccgcgtaggcgctcgttggtccagcagaggcggccgcccttgcgcgagcagaatggcggtagggggtctagctgcgtctcgtccggggggtctgcgtccacggtaaagaccccgggcagcaggcgcgcgtcgaagtagtctatcttgcatccttgcaagtctagcgcctgctgccatgcgcgggcggcaagcgcgcgctcgtatgggttgagtgggggaccccatggcatggggtgggtgagcgcggaggcgtacatgccgcaaatgtcgtaaacgtagaggggctctctgagtattccaagatatgtagggtagcatcttccaccgcggatgctggcgcgcacgtaatcgtatagttcgtgcgagggagcgaggaggtcgggaccgaggttgctacgggcgggctgctctgctcggaagactatctgcctgaagatggcatgtgagttggatgatatggttggacgctggaagacgttgaagctggcgtctgtgagacctaccgcgtcacgcacgaaggaggcgtaggagtcgcgcagcttgttgaccagctcggcggtgacctgcacgtctagggcgcagtagtccagggtttccttgatgatgtcatacttatcctgtcccttttttttccacagctcgcggttgaggacaaactcttcgcggtctttccagtactcttggatcggaaacccgtcggcctccgaacggtaagagcctagcatgtagaactggttgacggcctggtaggcgcagcatcccttttctacgggtagcgcgtatgcctgcgcggccttccggagcgaggtgtgggtgagcgcaaaggtgtccctgaccatgactttgaggtactggtatttgaagtcagtgtcgtcgcatccgccctgctcccagagcaaaaagtccgtgcgctttttggaacgcggatttggcagggcgaaggtgacatcgttgaagagtatctttcccgcgcgaggcataaagttgcgtgtgatgcggaagggtcccggcacctcggaacggttgttaattacctgggcggcgagcacgatctcgtcaaagccgttgatgttgtggcccacaatgtaaagttccaagaagcgcgggatgcccttgatggaaggcaattttttaagttcctcgtaggtgagctcttcaggggagctgagcccgtgctctgaaagggcccagtctgcaagatgagggttggaagcgacgaatgagctccacaggtcacgggccattagcatttgcaggtggtcgcgaaaggtcctaaactggcgacctatggccattttttctggggtgatgcagtagaaggtaagcgggtcttgttcccagcggtcccatccaaggttcgcggctaggtctcgcgcggcagtcactagaggctcatctccgccgaacttcatgaccagcatgaagggcacgagctgcttcccaaaggcccccatccaagtataggtctctacatcgtaggtgacaaagagacgctcggtgcgaggatgcgagccgatcgggaagaactggatctcccgccaccaattggaggagtggctattgatgtggtgaaagtagaagtccctgcgacgggccgaacactcgtgctggcttttgtaaaaacgtgcgcagtactggcagcggtgcacgggctgtacatcctgcacgaggttgacctgacgaccgcgcacaaggaagcagagtgggaatttgagcccctcgcctggcgggtttggctggtggtcttctacttcggctgcttgtccttgaccgtctggctgctcgaggggagttacggtggatcggaccaccacgccgcgcgagcccaaagtccagatgtccgcgcgcggcggtcggagcttgatgacaacatcgcgcagatgggagctgtccatggtctggagctcccgcggcgtcaggtcaggcgggagctcctgcaggtttacctcgcatagacgggtcagggcgcgggctagatccaggtgatacctaatttccaggggctggttggtggcggcgtcgatggcttgcaagaggccgcatccccgcggcgcgactacggtaccgcgcggcgggcggtgggccgcgggggtgtccttggatgatgcatctaaaagcggtgacgcgggcgagcccccggaggtagggggggctccggacccgccgggagagggggcaggggcacgtcggcgccgcgcgcgggcaggagctggtgctgcgcgcgtaggttgctggcgaacgcgacgacgcggcggttgatctcctgaatctggcgcctctgcgtgaagacgacgggcccggtgagcttgagcctgaaagagagttcgacagaatcaatttcggtgtcgttgacggcggcctggcgcaaaatctcctgcacgtctcctgagttgtcttgataggcgatctcggccatgaactgctcgatctcttcctcctggagatctccgcgtccggctcgctccacggtggcggcgaggtcgttggaaatgcgggccatgagctgcgagaaggcgttgaggcctccctcgttccagacgcggctgtagaccacgcccccttcggcatcgcgggcgcgcatgaccacctgcgcgagattgagctccacgtgccgggcgaagacggcgtagtttcgcaggcgctgaaagaggtagttgagggtggtggcggtgtgttctgccacgaagaagtacataacccagcgtcgcaacgtggattcgttgatatcccccaaggcctcaaggcgctccatggcctcgtagaagtccacggcgaagttgaaaaactgggagttgcgcgccgacacggttaactcctcctccagaagacggatgagctcggcgacagtgtcgcgcacctcgcgctcaaaggctacaggggcctcttcttcttcttcaatctcctcttccataagggcctccccttcttcttcttctggcggcggtgggggaggggggacacggcggcgacgacggcgcaccgggaggcggtcgacaaagcgctcgatcatctccccgcggcgacggcgcatggtctcggtgacggcgcggccgttctcgcgggggcgcagttggaagacgccgcccgtcatgtcccggttatgggttggcggggggctgccatgcggcagggatacggcgctaacgatgcatctcaacaattgttgtgtaggtactccgccgccgagggacctgagcgagtccgcatcgaccggatcggaaaacctctcgagaaaggcgtctaaccagtcacagtcgcaaggtaggctgagcaccgtggcgggcggcagcgggcggcggtcggggttgtttctggcggaggtgctgctgatgatgtaattaaagtaggcggtcttgagacggcggatggtcgacagaagcaccatgtccttgggtccggcctgctgaatgcgcaggcggtcggccatgccccaggcttcgttttgacatcggcgcaggtctttgtagtagtcttgcatgagcctttctaccggcacttcttcttctccttcctcttgtcctgcatctcttgcatctatcgctgcggcggcggcggagtttggccgtaggtggcgccctcttcctcccatgcgtgtgaccccgaagcccctcatcggctgaagcagggctaggtcggcgacaacgcgctcggctaatatggcctgctgcacctgcgtgagggtagactggaagtcatccatgtccacaaagcggtggtatgcgcccgtgttgatggtgtaagtgcagttggccataacggaccagttaacggtctggtgacccggctgcgagagctcggtgtacctgagacgcgagtaagccctcgagtcaaatacgtagtcgttgcaagtccgcaccaggtactggtatcccaccaaaaagtgcggcggcggctggcggtagaggggccagcgtagggtggccggggctccgggggcgagatcttccaacataaggcgatgatatccgtagatgtacctggacatccaggtgatgccggcggcggtggtggaggcgcgcggaaagtcgcggacgcggttccagatgttgcgcagcggcaaaaagtgctccatggtcgggacgctctggccggtcaggcgcgcgcaatcgttgacgctctaccgtgcaaaaggagagcctgtaagcgggcactcttccgtggtctggtggataaattcgcaagggtatcatggcggacgaccggggttcgagccccgtatccggccgtccgccgtgatccatgcggttaccgcccgcgtgtcgaacccaggtgtgcgacgtcagacaacgggggagtgctccttttggcttccttccaggcgcggcggctgctgcgctagcttttttggccactggccgcgcgcagcgtaagcggttaggctggaaagcgaaagcattaagtggctcgctccctgtagccggagggttattttccaagggttgagtcgcgggacccccggttcgagtctcggaccggccggactgcggcgaacgggggtttgcctccccgtcatgcaagaccccgcttgcaaattcctccggaaacagggacgagccccttttttgcttttcccagatgcatccggtgctgcggcagatgcgcccccctcctcagcagcggcaagagcaagagcagcggcagacatgcagggcaccctcccctcctcctaccgcgtcaggaggggcgacatccgcggttgacgcggcagcagatggtgattacgaacccccgcggcgccgggcccggcactacctggacttggaggagggcgagggcctggcgcggctaggagcgccctctcctgagcggtacccaagggtgcagctgaagcgtgatacgcgtgaggcgtacgtgccgcggcagaacctgtttcgcgaccgcgagggagaggagcccgaggagatgcgggatcgaaagttccacgcagggcgcgagctgcggcatggcctgaatcgcgagcggttgctgcgcgaggaggactttgagcccgacgcgcgaaccgggattagtcccgcgcgcgcacacgtggcggccgccgacctggtaaccgcatacgagcagacggtgaaccaggagattaactttcaaaaaagctttaacaaccacgtgcgtacgcttgtggcgcgcgaggaggtggctataggactgatgcatctgtgggactttgtaagcgcgctggagcaaaacccaaatagcaagccgctcatggcgcagctgttccttatagtgcagcacagcagggacaacgaggcattcagggatgcgctgctaaacatagtagagcccgagggccgctggctgctcgatttgataaacatcctgcagagcatagtggtgcaggagcgcagcttgagcctggctgacaaggtggccgccatcaactattccatgcttagcctgggcaagttttacgcccgcaagatataccataccccttacgttcccatagacaaggaggtaaagatcgaggggttctacatgcgcatggcgctgaaggtgcttaccttgagcgacgacctgggcgtttatcgcaacgagcgcatccacaaggccgtgagcgtgagccggcggcgcgagctcagcgaccgcgagctgatgcacagcctgcaaagggccctggctggcacgggcagcggcgatagagaggccgagtcctactttgacgcgggcgctgacctgcgctgggccccaagccgacgcgccctggaggcagctggggccggacctgggctggcggtggcacccgcgcgcgctggcaacgtcggcggcgtggaggaatatgacgaggacgatgagtacgagccagaggacggcgagtactaagcggtgatgtttctgatcagatgatgcaagacgcaacggacccggcggtgcgggcggcgctgcagagccagccgtccggccttaactccacggacgactggcgccaggtcatggaccgcatcatgtcgctgactgcgcgcaatcctgacgcgttccggcagcagccgcaggccaaccggctctccgcaattctggaagcggtggtcccggcgcgcgcaaaccccacgcacgagaaggtgctggcgatcgtaaacgcgctggccgaaaacagggccatccggcccgacgaggccggcctggtctacgacgcgctgcttcagcgcgtggctcgttacaacagcggcaacgtgcagaccaacctggaccggctggtgggggatgtgcgcgaggccgtggcgcagcgtgagcgcgcgcagcagcagggcaacctgggctccatggttgcactaaacgccttcctgagtacacagcccgccaacgtgccgcggggacaggaggactacaccaactttgtgagcgcactgcggctaatggtgactgagacaccgcaaagtgaggtgtaccagtctgggccagactattttttccagaccagtagacaaggcctgcagaccgtaaacctgagccaggctttcaaaaacttgcaggggctgtggggggtgcgggctcccacaggcgaccgcgcgaccgtgtctagcttgctgacgcccaactcgcgcctgttgctgctgctaatagcgcccttcacggacagtggcagcgtgtcccgggacacatacctaggtcacttgctgacactgtaccgcgaggccataggtcaggcgcatgtggacgagcatactttccaggagattacaagtgtcagccgcgcgctggggcaggaggacacgggcagcctggaggcaaccctaaactacctgctgaccaaccggcggcagaagatcccctcgttgcacagtttaaacagcgaggaggagcgcattttgcgctacgtgcagcagagcgtgagccttaacctgatgcgcgacggggtaacgcccagcgtggcgctggacatgaccgcgcgcaacatggaaccgggcatgtatgcctcaaaccggccgtttatcaaccgcctaatggactacttgcatcgcgcggccgccgtgaaccccgagtatttcaccaatgccatcttgaacccgcactggctaccgccccctggtttctacaccgggggattcgaggtgcccgagggtaacgatggattcctctgggacgacatagacgacagcgtgttttccccgcaaccgcagaccctgctagagttgcaacagcgcgagcaggcagaggcggcgctgcgaaaggaaagcttccgcaggccaagcagcttgtccgatctaggcgctgcggccccgcggtcagatgctagtagcccatttccaagcttgatagggtctcttaccagcactcgcaccacccgcccgcgcctgctgggcgaggaggagtacctaaacaactcgctgctgcagccgcagcgcgaaaaaaacctgcctccggcatttcccaacaacgggatagagagcctagtggacaagatgagtagatggaagacgtacgcgcaggagcacagggacgtgccaggcccgcgcccgcccacccgtcgtcaaaggcacgaccgtcagcggggtctggtgtgggaggacgatgactcggcagacgacagcagcgtcctggatttgggagggagtggcaacccgtttgcgcaccttcgccccaggctggggagaatgttttaaaaaaaaaaaagcatgatgcaaaataaaaaactcaccaaggccatggcaccgagcgttggttttcttgtattccccttagtatgcggcgcgcggcgatgtatgaggaaggtcctcctccctcctacgagagtgtggtgagcgcggcgccagtggcggcggcgctgggttctcccttcgatgctcccctggacccgccgtttgtgcctccgcggtacctgcggcctaccggggggagaaacagcatccgttactctgagttggcacccctattcgacaccacccgtgtgtacctggtggacaacaagtcaacggatgtggcatccctgaactaccagaacgaccacagcaactttctgaccacggtcattcaaaacaatgactacagcccgggggaggcaagcacacagaccatcaatcttgacgaccggtcgcactggggcggcgacctgaaaaccatcctgcataccaacatgccaaatgtgaacgagttcatgtttaccaataagtttaaggcgcgggtgatggtgtcgcgcttgcctactaaggacaatcaggtggagctgaaatacgagtgggtggagttcacgctgcccgagggcaactactccgagaccatgaccatagaccttatgaacaacgcgatcgtggagcactacttgaaagtgggcagacagaacggggttctggaaagcgacatcggggtaaagtttgacacccgcaacttcagactggggtttgaccccgtcactggtcttgtcatgcctggggtatatacaaacgaagccttccatccagacatcattttgctgccaggatgcggggtggacttcacccacagccgcctgagcaacttgttgggcatccgcaagcggcaacccttccaggagggctttaggatcacctacgatgatctggagggtggtaacattcccgcactgttggatgtggacgcctaccaggcgagcttgaaagatgacaccgaacagggcgggggtggcgcaggcggcagcaacagcagtggcagcggcgcggaagagaactccaacgcggcagccgcggcaatgcagccggtggaggacatgaacgatcatgccattcgcggcgacacctttgccacacgggctgaggagaagcgcgctgaggccgaagcagcggccgaagctgccgcccccgctgcgcaacccgaggtcgagaagcctcagaagaaaccggtgatcaaacccctgacagaggacagcaagaaacgcagttacaacctaataagcaatgacagcaccttcacccagtaccgcagctggtaccttgcatacaactacggcgaccctcagaccggaatccgctcatggaccctgctttgcactcctgacgtaacctgcggctcggagcaggtctactggtcgttgccagacatgatgcaagaccccgtgaccttccgctccacgcgccagatcagcaactttccggtggtgggcgccgagctgttgcccgtgcactccaagagcttctacaacgaccaggccgtctactcccaactcatccgccagtttacctctctgacccacgtgttcaatcgctttcccgagaaccagattttggcgcgcccgccagcccccaccatcaccaccgtcagtgaaaacgttcctgctctcacagatcacgggacgctaccgctgcgcaacagcatcggaggagtccagcgagtgaccattactgacgccagacgccgcacctgcccctacgtttacaaggccctgggcatagtctcgccgcgcgtcctatcgagccgcactttttgagcaagcatgtccatccttatatcgcccagcaataacacaggctggggcctgcgcttcccaagcaagatgtttggcggggccaagaagcgctccgaccaacacccagtgcgcgtgcgcgggcactaccgcgcgccctggggcgcgcacaaacgcggccgcactgggcgcaccaccgtcgatgacgccatcgacgcggtggtggaggaggcgcgcaactacacgcccacgccgccaccagtgtccacagtggacgcggccattcagaccgtggtgcgcggagcccggcgctatgctaaaatgaagagacggcggaggcgcgtagcacgtcgccaccgccgccgacccggcactgccgcccaacgcgcggcggcggccctgcttaaccgcgcacgtcgcaccggccgacgggcggccatgcgggccgctcgaaggctggccgcgggtattgtcactgtgccccccaggtccaggcgacgagcggccgccgcagcagccgcggccattagtgctatgactcagggtcgcaggggcaacgtgtattgggtgcgcgactcggttagcggcctgcgcgtgcccgtgcgcacccgccccccgcgcaactagattgcaagaaaaaactacttagactcgtactgttgtatgtatccagcggcggcggcgcgcaacgaagctatgtccaagcgcaaaatcaaagaagagatgctccaggtcatcgcgccggagatctatggccccccgaagaaggaagagcaggattacaagccccgaaagctaaagcgggtcaaaaagaaaaagaaagatgatgatgatgaacttgacgacgaggtggaactgctgcacgctaccgcgcccaggcgacgggtacagtggaaaggtcgacgcgtaaaacgtgttttgcgacccggcaccaccgtagtctttacgcccggtgagcgctccacccgcacctacaagcgcgtgtatgatgaggtgtacggcgacgaggacctgcttgagcaggccaacgagcgcctcggggagtttgcctacggaaagcggcataaggacatgctggcgttgccgctggacgagggcaacccaacacctagcctaaagcccgtaacactgcagcaggtgctgcccgcgcttgcaccgtccgaagaaaagcgcggcctaaagcgcgagtctggtgacttggcacccaccgtgcagctgatggtacccaagcgccagcgactggaagatgtcttggaaaaaatgaccgtggaacctgggctggagcccgaggtccgcgtgcggccaatcaagcaggtggcgccgggactgggcgtgcagaccgtggacgttcagatacccactaccagtagcaccagtattgccaccgccacagagggcatggagacacaaacgtccccggttgcctcagcggtggcggatgccgcggtgcaggcggtcgctgcggccgcgtccaagacctctacggaggtgcaaacggacccgtggatgtttcgcgtttcagccccccggcgcccgcgcggttcgaggaagtacggcgccgccagcgcgctactgcccgaatatgccctacatccttccattgcgcctacccccggctatcgtggctacacctaccgccccagaagacgagcaactacccgacgccgaaccaccactggaacccgccgccgccgtcgccgtcgccagcccgtgctggccccgatttccgtgcgcagggtggctcgcgaaggaggcaggaccctggtgctgccaacagcgcgctaccaccccagcatcgtttaaaagccggtctttgtggttcttgcagatatggccctcacctgccgcctccgtttcccggtgccgggattccgaggaagaatgcaccgtaggaggggcatggccggccacggcctgacgggcggcatgcgtcgtgcgcaccaccggcggcggcgcgcgtcgcaccgtcgcatgcgcggcggtatcctgcccctccttattccactgatcgccgcggcgattggcgccgtgcccggaattgcatccgtggccttgcaggcgcagagacactgattaaaaacaagttgcatgtggaaaaatcaaaataaaaagtctggactctcacgctcgcttggtcctgtaactattttgtagaatggaagacatcaactttgcgtctctggccccgcgacacggctcgcgcccgttcatgggaaactggcaagatatcggcaccagcaatatgagcggtggcgccttcagctggggctcgctgtggagcggcattaaaaatttcggttccaccgttaagaactatggcagcaaggcctggaacagcagcacaggccagatgctgagggataagttgaaagagcaaaatttccaacaaaaggtggtagatggcctggcctctggcattagcggggtggtggacctggccaaccaggcagtgcaaaataagattaacagtaagcttgatccccgccctcccgtagaggagcctccaccggccgtggagacagtgtctccagaggggcgtggcgaaaagcgtccgcgccccgacagggaagaaactctggtgacgcaaatagacgagcctccctcgtacgaggaggcactaaagcaaggcctgcccaccacccgtcccatcgcgcccatggctaccggagtgctgggccagcacacacccgtaacgctggacctgcctccccccgccgacacccagcagaaacctgtgctgccaggcccgaccgccgttgttgtaacccgtcctagccgcgcgtccctgcgccgcgccgccagcggtccgcgatcgttgcggcccgtagccagtggcaactggcaaagcacactgaacagcatcgtgggtctgggggtgcaatccctgaagcgccgacgatgcttctgaatagctaacgtgtcgtatgtgtgtcatgtatgcgtccatgtcgccgccagaggagctgctgagccgccgcgcgcccgctttccaagatggctaccccttcgatgatgccgcagtggtcttacatgcacatctcgggccaggacgcctcggagtacctgagccccgggctggtgcagtttgcccgcgccaccgagacgtacttcagcctgaataacaagtttagaaaccccacggtggcgcctacgcacgacgtgaccacagaccggtcccagcgtttgacgctgcggttcatccctgtggaccgtgaggatactgcgtactcgtacaaggcgcggttcaccctagctgtgggtgataaccgtgtgctggacatggcttccacgtactttgacatccgcggcgtgctggacaggggccctacttttaagccctactctggcactgcctacaacgccctggctcccaagggtgccccaaatccttgcgaatgggatgaagctgctactgctcttgaaataaacctagaagaagaggacgatgacaacgaagacgaagtagacgagcaagctgagcagcaaaaaactcacgtatttgggcaggcgccttattctggtataaatattacaaaggagggtattcaaataggtgtcgaaggtcaaacacctaaatatgccgataaaacatttcaacctgaacctcaaataggagaatctcagtggtacgaaactgaaattaatcatgcagctgggagagtccttaaaaagactaccccaatgaaaccatgttacggttcatatgcaaaacccacaaatgaaaatggagggcaaggcattcttgtaaagcaacaaaatggaaagctagaaagtcaagtggaaatgcaatttttctcaactactgaggcgaccgcaggcaatggtgataacttgactcctaaagtggtattgtacagtgaagatgtagatatagaaaccccagacactcatatttcttacatgcccactattaaggaaggtaactcacgagaactaatgggccaacaatctatgcccaacaggcctaattacattgcttttagggacaattttattggtctaatgtattacaacagcacgggtaatatgggtgttctggcgggccaagcatcgcagttgaatgctgttgtagatttgcaagacagaaacacagagctttcataccagcttttgcttgattccattggtgatagaaccaggtacttttctatgtggaatcaggctgttgacagctatgatccagatgttagaattattgaaaatcatggaactgaagatgaacttccaaattactgctttccactgggaggtgtgattaatacagagactcttaccaaggtaaaacctaaaacaggtcaggaaaatggatgggaaaaagatgctacagaattttcagataaaaatgaaataagagttggaaataattttgccatggaaatcaatctaaatgccaacctgtggagaaatttcctgtactccaacatagcgctgtatttgcccgacaagctaaagtacagtccttccaacgtaaaaatttctgataacccaaacacctacgactacatgaacaagcgagtggtggctcccgggttagtggactgctacattaaccttggagcacgctggtcccttgactatatggacaacgtcaacccatttaaccaccaccgcaatgctggcctgcgctaccgctcaatgttgctgggcaatggtcgctatgtgcccttccacatccaggtgcctcagaagttctttgccattaaaaacctccttctcctgccgggctcatacacctacgagtggaacttcaggaaggatgttaacatggttctgcagagctccctaggaaatgacctaagggttgacggagccagcattaagtttgatagcatttgcctttacgccaccttcttccccatggcccacaacaccgcctccacgcttgaggccatgcttagaaacgacaccaacgaccagtcctttaacgactatctctccgccgccaacatgctctaccctatacccgccaacgctaccaacgtgcccatatccatcccctcccgcaactgggcggctttccgcggctgggccttcacgcgccttaagactaaggaaaccccatcactgggctcgggctacgacccttattacacctactctggctctataccctacctagatggaaccttttacctcaaccacacctttaagaaggtggccattacctttgactcttctgtcagctggcctggcaatgaccgcctgcttacccccaacgagtttgaaattaagcgctcagttgacggggagggttacaacgttgcccagtgtaacatgaccaaagactggttcctggtacaaatgctagctaactacaacattggctaccagggcttctatatcccagagagctacaaggaccgcatgtactccttctttagaaacttccagcccatgagccgtcaggtggtggatgatactaaatacaaggactaccaacaggtgggcatcctacaccaacacaacaactctggatttgttggctaccttgcccccaccatgcgcgaaggacaggcctaccctgctaacttcccctatccgcttataggcaagaccgcagttgacagcattacccagaaaaagtttctttgcgatcgcaccctttggcgcatcccattctccagtaactttatgtccatgggcgcactcacagacctgggccaaaaccttctctacgccaactccgcccacgcgctagacatgacttttgaggtggatcccatggacgagcccacccttctttatgttttgtttgaagtctttgacgtggtccgtgtgcaccggccgcaccgcggcgtcatcgaaaccgtgtacctgcgcacgcccttctcggccggcaacgccacaacataaagaagcaagcaacatcaacaacagctgccgccatgggctccagtgagcaggaactgaaagccattgtcaaagatcttggttgtgggccatattttttgggcacctatgacaagcgctttccaggctttgtttctccacacaagctcgcctgcgccatagtcaatacggccggtcgcgagactgggggcgtacactggatggcctttgcctggaacccgcactcaaaaacatgctacctctttgagccctttggcttttctgaccagcgactcaagcaggtttaccagtttgagtacgagtcactcctgcgccgtagcgccattgcttcttcccccgaccgctgtataacgctggaaaagtccacccaaagcgtacaggggcccaactcggccgcctgtggactattctgctgcatgtttctccacgcctttgccaactggccccaaactcccatggatcacaaccccaccatgaaccttattaccggggtacccaactccatgctcaacagtccccaggtacagcccaccctgcgtcgcaaccaggaacagctctacagcttcctggagcgccactcgccctacttccgcagccacagtgcgcagattaggagcgccacttctttttgtcacttgaaaaacatgtaaaaataatgtactagagacactttcaataaaggcaaatgcttttatttgtacactctcgggtgattatttacccccacccttgccgtctgcgccgtttaaaaatcaaaggggttctgccgcgcatcgctatgcgccactggcagggacacgttgcgatactggtgtttagtgctccacttaaactcaggcacaaccatccgcggcagctcggtgaagttttcactccacaggctgcgcaccatcaccaacgcgtttagcaggtcgggcgccgatatcttgaagtcgcagttggggcctccgccctgcgcgcgcgagttgcgatacacagggttgcagcactggaacactatcagcgccgggtggtgcacgctggccagcacgctcttgtcggagatcagatccgcgtccaggtcctccgcgttgctcagggcgaacggagtcaactttggtagctgccttcccaaaaagggcgcgtgcccaggctttgagttgcactcgcaccgtagtggcatcaaaaggtgaccgtgcccggtctgggcgttaggatacagcgcctgcataaaagccttgatctgcttaaaagccacctgagcctttgcgccttcagagaagaacatgccgcaagacttgccggaaaactgattggccggacaggccgcgtcgtgcacgcagcaccttgcgtcggtgttggagatctgcaccacatttcggccccaccggttcttcacgatcttggccttgctagactgctccttcagcgcgcgctgcccgttttcgctcgtcacatccatttcaatcacgtgctccttatttatcataatgcttccgtgtagacacttaagctcgccttcgatctcagcgcagcggtgcagccacaacgcgcagcccgtgggctcgtgatgcttgtaggtcacctctgcaaacgactgcaggtacgcctgcaggaatcgccccatcatcgtcacaaaggtcttgttgctggtgaaggtcagctgcaacccgcggtgctcctcgttcagccaggtcttgcatacggccgccagagcttccacttggtcaggcagtagtttgaagttcgcctttagatcgttatccacgtggtacttgtccatcagcgcgcgcgcagcctccatgcccttctcccacgcagacacgatcggcacactcagcgggttcatcaccgtaatttcactttccgcttcgctgggctcttcctcttcctcttgcgtccgcataccacgcgccactgggtcgtcttcattcagccgccgcactgtgcgcttacctcctttgccatgcttgattagcaccggtgggttgctgaaacccaccatttgtagcgccacatcttctctttcttcctcgctgtccacgattacctctggtgatggcgggcgctcgggcttgggagaagggcgcttctttttcttcttgggcgcaatggccaaatccgccgccgaggtcgatggccgcgggctgggtgtgcgcggcaccagcgcgtcttgtgatgagtcttcctcgtcctcggactcgatacgccgcctcatccgcttttttgggggcgcccggggaggcggcggcgacggggacggggacgacacgtcctccatggttgggggacgtcgcgccgcaccgcgtccgcgctcgggggtggtttcgcgctgctcctcttcccgactggccatttccttctcctataggcagaaaaagatcatggagtcagtcgagaagaaggacagcctaaccgccccctctgagttcgccaccaccgcctccaccgatgccgccaacgcgcctaccaccttccccgtcgaggcacccccgcttgaggaggaggaagtgattatcgagcaggacccaggttttgtaagcgaagacgacgaggaccgctcagtaccaacagaggataaaaagcaagaccaggacaacgcagaggcaaacgaggaacaagtcgggcggggggacgaaaggcatggcgactacctagatgtgggagacgacgtgctgttgaagcatctgcagcgccagtgcgccattatctgcgacgcgttgcaagagcgcagcgatgtgcccctcgccatagcggatgtcagccttgcctacgaacgccacctattctcaccgcgcgtaccccccaaacgccaagaaaacggcacatgcgagcccaacccgcgcctcaacttctaccccgtatttgccgtgccagaggtgcttgccacctatcacatctttttccaaaactgcaagatacccctatcctgccgtgccaaccgcagccgagcggacaagcagctggccttgcggcagggcgctgtcatacctgatatcgcctcgctcaacgaagtgccaaaaatctttgagggtcttggacgcgacgagaagcgcgcggcaaacgctctgcaacaggaaaacagcgaaaatgaaagtcactctggagtgttggtggaactcgagggtgacaacgcgcgcctagccgtactaaaacgcagcatcgaggtcacccactttgcctacccggcacttaacctaccccccaaggtcatgagcacagtcatgagtgagctgatcgtgcgccgtgcgcagcccctggagagggatgcaaatttgcaagaacaaacagaggagggcctacccgcagttggcgacgagcagctagcgcgctggcttcaaacgcgcgagcctgccgacttggaggagcgacgcaaactaatgatggccgcagtgctcgttaccgtggagcttgagtgcatgcagcggttctttgctgacccggagatgcagcgcaagctagaggaaacattgcactacacctttcgacagggctacgtacgccaggcctgcaagatctccaacgtggagctctgcaacctggtctcctaccttggaattttgcacgaaaaccgccttgggcaaaacgtgcttcattccacgctcaagggcgaggcgcgccgcgactacgtccgcgactgcgtttacttatttctatgctacacctggcagacggccatgggcgtttggcagcagtgcttggaggagtgcaacctcaaggagctgcagaaactgctaaagcaaaacttgaaggacctatggacggccttcaacgagcgctccgtggccgcgcacctggcggacatcattttccccgaacgcctgcttaaaaccctgcaacagggtctgccagacttcaccagtcaaagcatgttgcagaactttaggaactttatcctagagcgctcaggaatcttgcccgccacctgctgtgcacttcctagcgactttgtgcccattaagtaccgcgaatgccctccgccgctttggggccactgctaccttctgcagctagccaactaccttgcctaccactctgacataatggaagacgtgagcggtgacggtctactggagtgtcactgtcgctgcaacctatgcaccccgcaccgctccctggtttgcaattcgcagctgcttaacgaaagtcaaattatcggtacctttgagctgcagggtccctcgcctgacgaaaagtccgcggctccggggttgaaactcactccggggctgtggacgtcggcttaccttcgcaaatttgtacctgaggactaccacgcccacgagattaggttctacgaagaccaatcccgcccgccaaatgcggagcttaccgcctgcgtcattacccagggccacattcttggccaattgcaagccatcaacaaagcccgccaagagtttctgctacgaaagggacggggggtttacttggacccccagtccggcgaggagctcaacccaatccccccgccgccgcagccctatcagcagcagccgcgggcccttgcttcccaggatggcacccaaaaagaagctgcagctgccgccgccacccacggacgaggaggaatactgggacagtcaggcagaggaggttttggacgaggaggaggaggacatgatggaagactgggagagcctagacgaggaagcttccgaggtcgaagaggtgtcagacgaaacaccgtcaccctcggtcgcattcccctcgccggcgccccagaaatcggcaaccggttccagcatggctacaacctccgctcctcaggcgccgccggcactgcccgttcgccgacccaaccgtagatgggacaccactggaaccagggccggtaagtccaagcagccgccgccgttagcccaagagcaacaacagcgccaaggctaccgctcatggcgcgggcacaagaacgccatagttgcttgcttgcaagactgtgggggcaacatctccttcgcccgccgctttcttctctaccatcacggcgtggccttcccccgtaacatcctgcattactaccgtcatctctacagcccatactgcaccggcggcagcggcagcggcagcaacagcagcggccacacagaagcaaaggcgaccggatagcaagactctgacaaagcccaagaaatccacagcggcggcagcagcaggaggaggagcgctgcgtctggcgcccaacgaacccgtatcgacccgcgagcttagaaacaggatttttcccactctgtatgctatatttcaacagagcaggggccaagaacaagagctgaaaataaaaaacaggtctctgcgatccctcacccgcagctgcctgtatcacaaaagcgaagatcagcttcggcgcacgctggaagacgcggaggctctcttcagtaaatactgcgcgctgactcttaaggactagtttcgcgccctttctcaaatttaagcgcgaaaactacgtcatctccagcggccacacccggcgccagcacctgtcgtcagcgccattatgagcaaggaaattcccacgccctacatgtggagttaccagccacaaatgggacttgcggctggagctgcccaagactactcaacccgaataaactacatgagcgcgggaccccacatgatatcccgggtcaacggaatccgcgcccaccgaaaccgaattctcttggaacaggcggctattaccaccacacctcgtaataaccttaatccccgtagttggcccgctgccctggtgtaccaggaaagtcccgctcccaccactgtggtacttcccagagacgcccaggccgaagttcagatgactaactcaggggcgcagcttgcgggcggctttcgtcacagggtgcggtcgcccgggcagggtataactcacctgacaatcagagggcgaggtattcagctcaacgacgagtcggtgagctcctcgcttggtctccgtccggacgggacatttcagatcggcggcgccggccgtccttcattcacgcctcgtcaggcaatcctaactctgcagacctcgtcctctgagccgcgctctggaggcattggaactctgcaatttattgaggagtttgtgccatcggtctactttaaccccttctcgggacctcccggccactatccggatcaatttattcctaactttgacgcggtaaaggactcggcggacggctacgactgaatgttaagtggagaggcagagcaactgcgcctgaaacacctggtccactgtcgccgccacaagtgctttgcccgcgactccggtgagttttgctactttgaattgcccgaggatcatatcgagggcccggcgcacggcgtccggcttaccgcccagggagagcttgcccgtagcctgattcgggagtttacccagcgccccctgctagttgagcgggacaggggaccctgtgttctcactgtgatttgcaactgtcctaaccttggattacatcaagatcctctagttataactagagtacccggggatcttattccctttaactaataaaaaaaaataataaagcatcacttacttaaaatcagttagcaaatttctgtccagtttattcagcagcacctccttgccctcctcccagctctggtattgcagcttcctcctggctgcaaactttctccacaatctaaatggaatgtcagtttcctcctgttcctgtccatccgcacccactatcttcatgttgttgcagatgaagcgcgcaagaccgtctgaagataccttcaaccccgtgtatccatatgacacggaaaccggtcctccaactgtgccttttcttactcctccctttgtatcccccaatgggtttcaagagagtccccctggggtactctctttgcgcctatccgaacctctagttacctccaatggcatgcttgcgctcaaaatgggcaacggcctctctctggacgaggccggcaaccttacctcccaaaatgtaaccactgtgagcccacctctcaaaaaaaccaagtcaaacataaacctggaaatatctgcacccctcacagttacctcagaagccctaactgtggctgccgccgcacctctaatggtcgcgggcaacacactcaccatgcaatcacaggccccgctaaccgtgcacgactccaaacttagcattgccacccaaggacccctcacagtgtcagaaggaaagctagccctgcaaacatcaggccccctcaccaccaccgatagcagtacccttactatcactgcctcaccccctctaactactgccactggtagcttgggcattgacttgaaagagcccatttatacacaaaatggaaaactaggactaaagtacggggctcctttgcatgtaacagacgacctaaacactttgaccgtagcaactggtccaggtgtgactattaataatacttccttgcaaactaaagttactggagccttgggttttgattcacaaggcaatatgcaacttaatgtagcaggaggactaaggattgattctcaaaacagacgccttatacttgatgttagttatccgtttgatgctcaaaaccaactaaatctaagactaggacagggccctctttttataaactcagcccacaacttggatattaactacaacaaaggcctttacttgtttacagcttcaaacaattccaaaaagcttgaggttaacctaagcactgccaaggggttgatgtttgacgctacagccatagccattaatgcaggagatgggcttgaatttggttcacctaatgcaccaaacacaaatcccctcaaaacaaaaattggccatggcctagaatttgattcaaacaaggctatggttcctaaactaggaactggccttagttttgacagcacaggtgccattacagtaggaaacaaaaataatgataagctaactttgtggaccacaccagctccatctcctaactgtagactaaatgcagagaaagatgctaaactcactttggtcttaacaaaatgtggcagtcaaatacttgctacagtttcagttttggctgttaaaggcagtttggctccaatatctggaacagttcaaagtgctcatcttattataagatttgacgaaaatggagtgctactaaacaattccttcctggacccagaatattggaactttagaaatggagatcttactgaaggcacagcctatacaaacgctgttggatttatgcctaacctatcagcttatccaaaatctcacggtaaaactgccaaaagtaacattgtcagtcaagtttacttaaacggagacaaaactaaacctgtaacactaaccattacactaaacggtacacaggaaacaggagacacaactccaagtgcatactctatgtcattttcatgggactggtctggccacaactacattaatgaaatatttgccacatcctcttacactttttcatacattgcccaagaataaagaatcgtttgtgttatgtttcaacgtgtttatttttcaattgcagaaaatttcaagtcatttttcattcagtagtatagccccaccaccacatagcttatacagatcaccgtaccttaatcaaactcacagaaccctagtattcaacctgccacctccctcccaacacacagagtacacagtcctttctccccggctggccttaaaaagcatcatatcatgggtaacagacatattcttaggtgttatattccacacggtttcctgtcgagccaaacgctcatcaagtgatattaataaactccccgggcagctcacttaagttcatgtcgctgtccagctgctgagccacaggctgctgtccaacttgcggttgcttaacgggcggcgaaggagaagtccacgcctacatggggggagagtcataatcgtgcatcaggatagggcggtggtgctgcagcagcgcgcgaataaactgctgccgccgccgctccgtcctgcaggaatacaacatggcagtggtctcctcagcgatgattcgcaccgcccgcagcataaggcgcttgtcctccgggcacagcagcgcaccctgatctcacttaaatcagcacagtaactgcagcacagcaccacaatattgttcaaaatcccacagtgcaaggcgctgtatccaaagctcatggcggggaccacagaacccacgtggccatcataccacaagcgcaggtagattaagtggcgacccctcataaacacgctggacataaacattacctcttttggcatgttgtaattcaccacctcccggtaccatataaacctctgattaaacatggcgccatccaccaccatcctaaaccagctggccaaaacctgccccgccgggntatacactgcagggaaccgggacttggacaatgacaagtgggagagcccaggactcgtaaccatggatcatcatgctcgtcatgatatcaatgttggcacaacacaggcacacgtgcatacacttcctcaggattacaagctcctcccgcgttagaaccatatcccagggaacaacccattcctgaatcagcgtaaatcccacactgcagggaagacctcgcacgtaactcacgttgtgcattgtcaaagtgttacattcgggcagcagcggatgatcctccagtatggtagcgcgggtttctgtctcaaaaggaggtagacgatccctactgtacggagtgcgccgagacaaccgagatcgtgttggtcgtagtgtcatgccaaatggaacgccggacgtagtcatatttcctgaagcaaaaccaggtgcgggcgtgacaaacagatctgcgtctccggtctcgccgcttagatcgctctgtgtagtagttgtagtatatccactctctcaaagcatccaggcgccccctggcttcgggttctatgtaaactccttcatgcgccgctgccctgataacatccaccaccgcagaataagccacacccagccaacctacacattcgttctgcgagtcacacacgggaggagcgggaagagctggaagaaccatgtttttttttttattccaaaagattatccaaaacctcaaaatgaagatctattaagtgaacgcgctcccctccggtggcgtggtcaaactctacagccaaagaacagataatggcatttgtaagatgttgcacaatggcttccaaaaggcaaacggccctcacgtccaagtggacgtaaaggctaaacccttcagggtgaatctcctctataaacattccagcaccttcaaccatgcccaaataattctcatctcgccaccttctcaatatatctctaagcaaatcccgaatatttaagtccgggccattgtaaaaaatttggctccagagcgccctccaccttcagcctcaagcagcgaatcatgattgcaaaaattcaggttcctcacagacctgtataagattcaaaagcggaacattaacaaaaataccgcgatcccgtaggtcccttcgcagggccagctgaacataatcgtgcaggtctgcacggaccagcgcggccacttccccgccaggaaccatgacaaaagaacccacactgattatgacacgcatactcggagctatgctaaccagcgtagccccgatgtaagcttgttgcatgggcggcgatataaaatgcaaggtgctgctcaaaaaatcaggcaaagcctcgcgcaaaaaagaaagcacatcgtagtcatgctcatgcagataaaggcaggtaagctccggaaccaccacagaaaaagacaccatttttctctcaaacatgtctgcgggtttctgcataaacacaaaataaaataacaaaaaaacatttaaacattagaagcctgtcttacaacaggaaaaacaacccttataagcataagacggactacggccatgccggcgtgaccgtaaaaaaactggtcaccgtgattaaaaagcaccaccgacagctcctcggtcagtccggagtcataatgtaagactcggtaaacacatcaggttgattcacatcggtcagtgttaaaaagcgaccgaaatagccngggggaatacaatacccgcaggcgtagagacaacattacagcccccataggaggtataacaaaattaataggagagaaaaacacataaacacctgaaaaaccctcctgcctaggcaaaatagcaccctcccgctccagaacaacatacagcgcttccacagcggcagccataacagtcagccttaccagtaaaaaagaaaacctattaaaaaaacaccactcgacacggcaccagctcaatcagtcacagtgtaaaaaagggccaagtgcagagcgagtatatataggactaaaaaatgacggtaacggttaaagtccacaaaaaacacccagaaaaccgcacgcgaacctacgcccagaaacgaaagccaaaaaacccacaacttcctcaaatcgtcacttccgttttcccacgttacgtcacttcccattttaagaaaactacaattcccaacacatacaagttactccgccctaaaacctacgtcacccgccccgttcccacgccccgcgccacgtcacaaactccaccccctcattatcatattggcttcaatccaaaataaggtatattattgatgatg

SEQ ID NO: 11 - DNA, 6253 bp, Artificial Sequence
  Example starter rAAV vector
  misc_feature 19..161: /note="TR"
  promoter 172..766: /note="Pcmv"
  misc_feature 763..942: /note="SV40 SD, SA"
  gene 988..1701: /gene="GFP gene"
  polyA_site 1712..1910: /note="SV40 polyA"
  enhancer 1922..2057: /note="PYF441 enhancer"
  misc_feature 2058..2186: /note="HSV-tk"
  gene 2198..3000: /gene="neoR"
  polyA_site 3010..3248: /note="bGH poly A"
  misc_feature 3259..3401: /note="TR"
  misc_feature 3850..4075: /note="ColE1ori"
  misc_feature 4325..5325: /note="ApR"
  misc_feature 5729..6188: /note="f1+ origin"
ggggggggggggggggggttggccactccctctctgcgcgctcgctcgctcactgaggccgggcgaccaaaggtcgcccgacgcccgggctttgcccgggcggcctcagtgagcgagcgagcgcgcagagagggagtggccaactccatcactaggggttcctagatctgaattcggtacccgttacataacttacggtaaatggcccgcctggctgaccgcccaacgacccccgcccattgacgtcaataatgacgtatgttcccatagtaacgccaatagggactttccattgacgtcaatgggtggagtatttacggtaaactgcccacttggcagtacatcaagtgtatcatatgccaagtacgccccctattgacgtcaatgacggtaaatggcccgcctggcattatgcccagtacatgaccttatgggactttcctacttggcagtacatctacgtattagtcatcgctattaccatggtgatgcggttttggcagtacatcaatgggcgtggatagcggtttgactcacggggatttccaagtctccaccccattgacgtcaatgggagtttgttttggcaccaaaatcaacgggactttccaaaatgtcgtaacaactccgccccattgacgcaaatgggcggtaggcgtgtacggtgggaggtctatataagcagagctcgtttagtgaaccgtcagatcgcctggagacgccatccacgctgttttgacctccatagaagacaccgggaccgatccagcctccggactctagaggatccggtactcgaggaactgaaaaaccagaaagttaactggtaagtttagtctttttgtcttttatttcaggtcccggatccggtggtggtgcaaatcaaagaactgctcctcagtggatgttgcctttacttctaggcctgtacggaagtgttacttctgctctaaaagctgcggaattgtacccgcggccgccgccaccatgagcaagggcgaggaactgttcactggcgtggtcccaattctcgtggaactggatggcgatgtgaatgggcacaaattttctgtcagcggagagggtgaaggtgatgccacatacggaaagctcaccctgaaattcatctgcaccactggaaagctccctgtgccatggccaacactggtcactaccctgacctatggcgtgcagtgcttttccagatacccagaccatatgaagcagcatgactttttcaagagcgccatgcccgagggctatgtgcaggagagaaccatctttttcaaagatgacgggaactacaagacccgcgctgaagtcaagttcgaaggtgacaccctggtgaatagaatcgagctgaagggcattgactttaaggaggatggaaacattctcggccacaagctggaatacaactataactcccacaatgtgtacatcatggccgacaagcaaaagaatggcatcaaggtcaacttcaagatcagacacaacattgaggatggatccgtgcagctggccgaccattatcaacagaacactccaatcggcgacggccctgtgctcctcccagacaaccattacctgtccacccagtctgccctgtctaaagatcccaacgaaaagagagaccacatggtcctgctggagtttgtgaccgctgctgggatcacacatggcatggacgagctgtacaagtgagcggccgcggggatccagacatgataagatacattgatgagtttggacaaaccacaactagaatgcagtgaaaaaaatgctttatttgtgaaatttgtgatgctattgctttatttgtaaccattataagctgcaataaacaagttaacaacaacaattgcattcattttatgtttcaggttcagggggaggtgtgggaggttttttagtcgacctcgagcagtgtggttttgcaagaggaagcaaaaagcctctccacccaggcctggaatgtttccacccaagtcgaaggcagtgtggttttgcaagaggaagcaaaaagcctctccacccaggcctggaatgtttccacccaatgtcgagcaaccccgcccagcgtcttgtcattggcgaattcgaacacgcagatgcagtcggggcggcgcggtcccaggtccacttcgcatattaaggtgacgcgtgtggcctcgaacaccgagcgaccctgcagccaatatgggatcggccattgaacaagatggattgcacgcaggttctccggccgcttgggtggagaggctattcggctatgactgggcacaacagacaatcggctgctctgatgccgccgtgttccggctgtcagcgcaggggcgcccggttctttttgtcaagaccgacctgtccggtgccctgaatgaactgcaggacgaggcagcgcggctatcgtggctggccacgacgggcgttccttgcgcagctgtgctcgacgttgtcactgaagcgggaagggactggctgctattgggcgaagtgccggggcaggatctcctgtcatctcaccttgctcctgccgagaaagtatccatcatggctgatgcaatgcggcggctgcatacgcttgatccggctacctgcccattcgaccaccaagcgaaacatcgcatcgagcgagcacgtactcggatggaagccggtcttgtcgatcaggatgatctggacgaagagcatcaggggctcgcgccagccgaactgttcgccaggctcaaggcgcgcatgcccgacggcgaggatctcgtcgtgacccatggcgatgcctgcttgccgaatatcatggtggaaaatggccgcttttctggattcatcgactgtggccggctgggtgtggcggaccgctatcaggacatagcgttggctacccgtgatattgctgaagagcttggcggcgaatgggctgaccgcttcctcgtgctttacggtatcgccgctcccgattcgcagcgcatcgccttctatcgccttcttgacgagttcttctgaggggatccgtcgactagagctcgctgatcagcctcgactgtgccttctagttgccagccatctgttgtttgcccctcccccgtgccttccttgaccctggaaggtgccactcccactgtcctttcctaataaaatgaggaaattgcatcgcattgtctgagtaggtgtcattctattctggggggtggggtggggcaggacagcaagggggaggattgggaagacaatagcaggcatgctggggagagatctaggaacccctagtgatggagttggccactccctctctgcgcgctcgctcgctcactgaggccgcccgggcaaagcccgggcgtcgggcgacctttggtcgcccggcctcagtgagcgagcgagcgcgcagagagggagtggccaacccccccccccccccccctgcagccctgcattaatgaatcggccaacgcgcggggagaggcggtttgcgtattgggcgctcttccgcttcctcgctcactgactcgctgcgctcggtcgttcggctgcggcgagcggtatcagctcactcaaaggcggtaatacggttatccacagaatcaggggataacgcaggaaagaacatgtgagcaaaaggccagcaaaaggccaggaaccgtaaaaaggccgcgttgctggcgtttttccataggctccgcccccctgacgagcatcacaaaaatcgacgctcaagtcagaggtggcgaaacccgacaggactataaagataccaggcgtttccccctggaagctccctcgtgcgctctcctgttccgaccctgccgcttaccggatacctgtccgcctttctcccttcgggaagcgtggcgctttctcaatgctcacgctgtaggtatctcagttcggtgtaggtcgttcgctccaagctgggctgtgtgcacgaaccccccgttcagcccgaccgctgcgccttatccggtaactatcgtcttgagtccaacccggtaagacacgacttatcgccactggcagcagccactggtaacaggattagcagagcgaggtatgtaggcggtgctacagagttcttgaagtggtggcctaactacggctacactagaaggacagtatttggtatctgcgctctgctgaagccagttaccttcggaaaaagagttggtagctcttgatccggcaaacaaaccaccgctggtagcggtggtttttttgtttgcaagcagcagattacgcgcagaaaaaaaggatctcaagaagatcctttgatcttttctacggggtctgacgctcagtggaacgaaaactcacgttaagggattttggtcatgagattatcaaaaaggatcttcacctagatccttttaaattaaaaatgaagttttaaatcaatctaaagtatatatgagtaaacttggtctgacagttaccaatgcttaatcagtgaggcacctatctcagcgatctgtctatttcgttcatccatagttgcctgactccccgtcgtgtagataactacgatacgggagggcttaccatctggccccagtgctgcaatgataccgcgagacccacgctcaccggctccagatttatcagcaataaaccagccagccggaagggccgagcgcagaagtggtcctgcaactttatccgcctccatccagtctattaattgttgccgggaagctagagtaagtagttcgccagttaatagtttgcgcaacgttgttgccattgctacaggcatcgtggtgtcacgctcgtcgtttggtatggcttcattcagctccggttcccaacgatcaaggcgagttacatgatcccccatgttgtgcaaaaaagcggttagctccttcggtcctccgatcgttgtcagaagtaagttggccgcagtgttatcactcatggttatggcagcactgcataattctcttactgtcatgccatccgtaagatgcttttctgtgactggtgagtactcaaccaagtcattctgagaatagtgtatgcggcgaccgagttgctcttgcccggcgtcaatacgggataataccgcgccacatagcagaactttaaaagtgctcatcattggaaaacgttcttcggggcgaaaactctcaaggatcttaccgctgttgagatccagttcgatgtaacccactcgtgcacccaactgatcttcagcatcttttactttcaccagcgtttctgggtgagcaaaaacaggaaggcaaaatgccgcaaaaaagggaataagggcgacacggaaatgttgaatactcatactcttcctttttcaatattattgaagcatttatcagggttattgtctcatgagcggatacatatttgaatgtatttagaaaaataaacaaataggggttccgcgcacatttccccgaaaagtgccacctgacgtctaagaaaccattattatcatgacattaacctataaaaataggcgtatcacgaggccctttcgtctcgcgcgtttcggtgatgacggtgaaaacctctgacacatgcagctcccggagacggtcacagcttgtctgtaagcggatgccgggagcagacaagcccgtcagggcgcgtcagcgggtgttggcgggtgtcggggctggcttaactatgcggcatcagagcagattgtactgagagtgcaccatatgcggtgtgaaataccgcacagatgcgtaaggagaaaataccgcatcaggaaattgtaaacgttaatattttgttaaaattcgcgttaaatttttgttaaatcagctcattttttaaccaataggccgaaatcggcaaaatcccttataaatcaaaagaatagaccgagatagggttgagtgttgttccagtttggaacaagagtccactattaaagaacgtggactccaacgtcaaagggcgaaaaaccgtctatcagggcgatggcccactacgtgaaccatcaccctaatcaagttttttggggtcgaggtgccgtaaagcactaaatcggaaccctaaagggagcccccgatttagagcttgacggggaaagccggcgaacgtggcgagaaaggaagggaagaaagcgaaaggagcgggcgctagggcgctggcaagtgtagcggtcacgctgcgcgtaaccaccacacccgccgcgcttaatgcgccgctacagggcgcgtcgcgccattcgccattcaggctacgcaactgttgggaagggcgatcggtgcgggcctcttcgctattacgccaggctgca

SEQ ID NO: 12 - DNA, 280 bp, Adeno-associated virus - 2
  Minimal RIS-Ad
aaagggtggagccaagaaaagacccgcccccagtgacgcagatataagtgagcccaaacgggtgcgcgagtcagttgcgcagccatcgacgtcagacgcggaagcttcgatcaactacgcagacaggtaccaaaacaaatgttctcgtcacgtgggcatgaatctgatgctgtttccctgcagacaatgcgagagaatgaatcagaattcaaatatctgcttcactcacggacagaaagactgtttagagtgctttcccgtgtcagaatctcaacccgtt

SEQ ID NO: 13 - DNA, 280 bp, Artificial Sequence
  Recoded minimal RIS-Ad
gaaggggggggccaaaaagcgccctgcaccttccgacgccgacatttccgagccaaagagagtgcgtgagagtgtggcccaaccctccaccagtgatgccgaggcctccattaattatgccgaccgctatcagaataagtgctcaaggcatgtcgggatgaacctgatgctgttcccatgccgccagtgcgagcgcatgaaccagaacagcaacatttgttttacccacgggcagaaggattgcctggaatgcttcccggtcagcgagtcacagccggtg

SEQ ID NO: 14 - protein, 735 aa, Adeno-associated virus - 2 [sequence omitted]